European Patent Application EP 4 389 758 A1, published June 26, 2024. Title: Human transferrin receptor binding peptide. Applicant: PeptiDream INC. Application JP. The sequence listing filed with the application follows.

SEQUENCE LISTING (253 sequences)

SEQ ID NO: 1 - protein, 15 aa, synthetic construct
  REGION 1..15: note = Synthesized polypeptide
  MOD_RES 3: note = METHYLATION
  BINDING 11: note = MePEG4c
  MOD_RES 14: note = METHYLATION
AVFVWNYYIIKRFYC

SEQ ID NO: 2 - protein, 15 aa, synthetic construct
  REGION 1..15: note = Synthesized polypeptide
  MOD_RES 3: note = METHYLATION
  BINDING 12: note = MePEG4c
  MOD_RES 14: note = METHYLATION
AVFVWNYYIIRKFYC

SEQ ID NO: 3 - protein, 15 aa, synthetic construct
  REGION 1..15: note = Synthesized polypeptide
  SITE 3: note = MISC_FEATURE - Xaa is MeF4F
  SITE 5: note = MISC_FEATURE - Xaa is W5C
  MOD_RES 11: note = METHYLATION
  BINDING 12: note = MePEG4c
  MOD_RES 14: note = METHYLATION
AVXVXNYYIIRKFYC

SEQ ID NO: 4 - protein, 15 aa, synthetic construct
  REGION 1..15: note = Synthesized polypeptide
  SITE 3: note = MISC_FEATURE - Xaa is MeF4F
  SITE 5: note = MISC_FEATURE - Xaa is W5C
  SITE 8: note = MISC_FEATURE - Xaa is F4OMe
  MOD_RES 11: note = METHYLATION
  BINDING 12: note = MePEG4c
  MOD_RES 14: note = METHYLATION
AVXVXNYXIIRKFYC

SEQ ID NO: 5 - protein, 15 aa, synthetic construct
  REGION 1..15: note = Synthesized polypeptide
  SITE 3: note = MISC_FEATURE - Xaa is MeF4F
  MOD_RES 5: note = METHYLATION
  BINDING 11: note = MePEG4c
  SITE 12: note = MISC_FEATURE - Xaa is dr
  MOD_RES 14: note = METHYLATION
AVXVWNYYIIKXFYC

SEQ ID NO: 6 - protein, 15 aa, synthetic construct
  REGION 1..15: note = Synthesized polypeptide
  SITE 3: note = MISC_FEATURE - Xaa is MeF4F
  MOD_RES 5: note = METHYLATION
  SITE 8: note = MISC_FEATURE - Xaa is F4OMe
  BINDING 11: note = MePEG4c
  SITE 12: note = MISC_FEATURE - Xaa is dr
  MOD_RES 14: note = METHYLATION
AVXVWNYXIIKXFYC

SEQ ID NO: 7 - protein, 15 aa, synthetic construct
  REGION 1..15: note = Synthesized polypeptide
  SITE 3: note = MISC_FEATURE - Xaa is MeF4F
  MOD_RES 5: note = METHYLATION
  MOD_RES 11: note = METHYLATION
  BINDING 12: note = MePEG4c
  MOD_RES 14: note = METHYLATION
AVXVWNYYIIRKFYC

SEQ ID NO: 8 - protein, 15 aa, synthetic construct
  REGION 1..15: note = Synthesized polypeptide
  SITE 3: note = MISC_FEATURE - Xaa is MeF4F
  MOD_RES 5: note = METHYLATION
  SITE 8: note = MISC_FEATURE - Xaa is F4OMe
  MOD_RES 11: note = METHYLATION
  BINDING 12: note = MePEG4c
  MOD_RES 14: note = METHYLATION
AVXVWNYXIIRKFYC

SEQ ID NO: 9 - protein, 15 aa, synthetic construct
  REGION 1..15: note = Synthesized polypeptide
  MOD_RES 3: note = METHYLATION
  SITE 6: note = MISC_FEATURE - Xaa is Ndm
  MOD_RES 14: note = METHYLATION
AVFVWXYYIIRRYYC

SEQ ID NO: 10 - protein, 15 aa, synthetic construct
  REGION 1..15: note = Synthesized polypeptide
  MOD_RES 1: note = METHYLATION
  SITE 3: note = MISC_FEATURE - Xaa is MeF3C
  MOD_RES 5: note = METHYLATION
  SITE 8: note = MISC_FEATURE - Xaa is F4OMe
  SITE 12: note = MISC_FEATURE - Xaa is da
  MOD_RES 14: note = METHYLATION
AVXVWNYXIIRXFYC

SEQ ID NO: 11 - protein, 15 aa, synthetic construct
  REGION 1..15: note = Synthesized polypeptide
  SITE 3: note = MISC_FEATURE - Xaa is MeF3C
  SITE 8: note = MISC_FEATURE - Xaa is F4OMe
  MOD_RES 14: note = METHYLATION
AVXVWNYXIIRRFYC

SEQ ID NO: 12 - protein, 15 aa, synthetic construct
  REGION 1..15: note = Synthesized polypeptide
  SITE 3: note = MISC_FEATURE - Xaa is MeF3C
  SITE 8: note = MISC_FEATURE - Xaa is F4OMe
  MOD_RES 14: note = METHYLATION
AVXVWNYXIIKRFYC

SEQ ID NO: 13 - protein, 15 aa, synthetic construct
  REGION 1..15: note = Synthesized polypeptide
  MOD_RES 3: note = METHYLATION
  MOD_RES 14: note = METHYLATION
AVFVWNYYIIRRYYC

SEQ ID NO: 14 - protein, 15 aa, synthetic construct
  REGION 1..15: note = Synthesized polypeptide
  MOD_RES 3: note = METHYLATION
  SITE 12: note = MISC_FEATURE - Xaa is dr
  MOD_RES 14: note = METHYLATION
AVFVWNYYIIRXFYC

SEQ ID NO: 15 - protein, 15 aa, synthetic construct
  REGION 1..15: note = Synthesized polypeptide
  MOD_RES 3: note = METHYLATION
  SITE 8: note = MISC_FEATURE - Xaa is F4OMe
  SITE 12: note = MISC_FEATURE - Xaa is dr
  MOD_RES 14: note = METHYLATION
AVFVWNYXIIRXFYC

SEQ ID NO: 16 - protein, 15 aa, synthetic construct
  REGION 1..15: note = Synthesized polypeptide
  MOD_RES 3: note = METHYLATION
  MOD_RES 11: note = METHYLATION
  MOD_RES 14: note = METHYLATION
AVFVWNYYIIRRFYC

SEQ ID NO: 17 - protein, 15 aa, synthetic construct
  REGION 1..15: note = Synthesized polypeptide
  MOD_RES 3: note = METHYLATION
  SITE 8: note = MISC_FEATURE - Xaa is F4OMe
  MOD_RES 11: note = METHYLATION
  MOD_RES 14: note = METHYLATION
AVFVWNYXIIRRFYC

SEQ ID NO: 18 - protein, 15 aa, synthetic construct
  REGION 1..15: note = Synthesized polypeptide
  MOD_RES 3: note = METHYLATION
  SITE 5: note = MISC_FEATURE - Xaa is W5C
  MOD_RES 14: note = METHYLATION
AVFVXNYYIIRRFYC

SEQ ID NO: 19 - protein, 15 aa, synthetic construct
  REGION 1..15: note = Synthesized polypeptide
  MOD_RES 3: note = METHYLATION
  SITE 5: note = MISC_FEATURE - Xaa is W5C
  SITE 8: note = MISC_FEATURE - Xaa is F4OMe
  MOD_RES 14: note = METHYLATION
AVFVXNYXIIRRFYC

SEQ ID NO: 20 - protein, 15 aa, synthetic construct
  REGION 1..15: note = Synthesized polypeptide
  MOD_RES 3: note = METHYLATION
  SITE 5: note = MISC_FEATURE - Xaa is W5C
  SITE 12: note = MISC_FEATURE - Xaa is dr
  MOD_RES 14: note = METHYLATION
AVFVXNYYIIRXFYC

SEQ ID NO: 21 - protein, 15 aa, synthetic construct
  REGION 1..15: note = Synthesized polypeptide
  MOD_RES 3: note = METHYLATION
  SITE 5: note = MISC_FEATURE - Xaa is W5C
  SITE 8: note = MISC_FEATURE - Xaa is F4OMe
  SITE 12: note = MISC_FEATURE - Xaa is dr
  MOD_RES 14: note = METHYLATION
AVFVXNYXIIRXFYC

SEQ ID NO: 22 - protein, 15 aa, synthetic construct
  REGION 1..15: note = Synthesized polypeptide
  SITE 3: note = MISC_FEATURE - Xaa is MeF4F
  SITE 5: note = MISC_FEATURE - Xaa is W5C
  MOD_RES 14: note = METHYLATION
AVXVXNYYIIRRFYC

SEQ ID NO: 23 - protein, 15 aa, synthetic construct
  REGION 1..15: note = Synthesized polypeptide
  SITE 3: note = MISC_FEATURE - Xaa is MeF4F
  SITE 5: note = MISC_FEATURE - Xaa is W5C
  SITE 8: note = MISC_FEATURE - Xaa is F4OMe
  MOD_RES 14: note = METHYLATION
AVXVXNYXIIRRFYC

SEQ ID NO: 24 - protein, 15 aa, synthetic construct
  REGION 1..15: note = Synthesized polypeptide
  SITE 3: note = MISC_FEATURE - Xaa is MeF4F
  SITE 5: note = MISC_FEATURE - Xaa is W5C
  SITE 12: note = MISC_FEATURE - Xaa is dr
  MOD_RES 14: note = METHYLATION
AVXVXNYYIIRXFYC

SEQ ID NO: 25 - protein, 15 aa, synthetic construct
  REGION 1..15: note = Synthesized polypeptide
  SITE 3: note = MISC_FEATURE - Xaa is MeF4F
  SITE 5: note = MISC_FEATURE - Xaa is W5C
  MOD_RES 11: note = METHYLATION
  SITE 12: note = MISC_FEATURE - Xaa is dr
  MOD_RES 14: note = METHYLATION
AVXVXNYYIIRXFYC

SEQ ID NO: 26 - protein, 15 aa, synthetic construct
  REGION 1..15: note = Synthesized polypeptide
  SITE 3: note = MISC_FEATURE - Xaa is MeF4F
  SITE 5: note = MISC_FEATURE - Xaa is W5C
  SITE 8: note = MISC_FEATURE - Xaa is F4OMe
  SITE 12: note = MISC_FEATURE - Xaa is dr
  MOD_RES 14: note = METHYLATION
AVXVXNYXIIRXFYC

SEQ ID NO: 27 - protein, 15 aa, synthetic construct
  REGION 1..15: note = Synthesized polypeptide
  SITE 3: note = MISC_FEATURE - Xaa is MeF4F
  SITE 5: note = MISC_FEATURE - Xaa is W5C
  SITE 8: note = MISC_FEATURE - Xaa is F4OMe
  MOD_RES 11: note = METHYLATION
  SITE 12: note = MISC_FEATURE - Xaa is dr
  MOD_RES 14: note = METHYLATION
AVXVXNYXIIRXFYC

SEQ ID NO: 28 - protein, 15 aa, synthetic construct
  REGION 1..15: note = Synthesized polypeptide
  SITE 3: note = MISC_FEATURE - Xaa is MeF4F
  MOD_RES 5: note = METHYLATION
  SITE 12: note = MISC_FEATURE - Xaa is dr
  MOD_RES 14: note = METHYLATION
AVXVWNYYIIRXFYC

SEQ ID NO: 29 - protein, 15 aa, synthetic construct
  REGION 1..15: note = Synthesized polypeptide
  SITE 3: note = MISC_FEATURE - Xaa is MeF4F
  MOD_RES 5: note = METHYLATION
  SITE 8: note = MISC_FEATURE - Xaa is F4OMe
  SITE 12: note = MISC_FEATURE - Xaa is dr
  MOD_RES 14: note = METHYLATION
AVXVWNYXIIRXFYC

SEQ ID NO: 30 - protein, 15 aa, synthetic construct
  REGION 1..15: note = Synthesized polypeptide
  SITE 3: note = MISC_FEATURE - Xaa is MeF4F
  MOD_RES 5: note = METHYLATION
  SITE 8: note = MISC_FEATURE - Xaa is F4OMe
  MOD_RES 11: note = METHYLATION
  SITE 12: note = MISC_FEATURE - Xaa is dr
  MOD_RES 14: note = METHYLATION
AVXVWNYXIIRXFYC

SEQ ID NO: 31 - protein, 15 aa, synthetic construct
  REGION 1..15: note = Synthesized polypeptide
  SITE 3: note = MISC_FEATURE - Xaa is MeF3C
  SITE 8: note = MISC_FEATURE - Xaa is F4OMe
  MOD_RES 14: note = METHYLATION
AVXVWNYXIIRRFYC

SEQ ID NO: 32 - protein, 15 aa, synthetic construct
  REGION 1..15: note = Synthesized polypeptide
  SITE 3: note = MISC_FEATURE - Xaa is MeF3C
  SITE 8: note = MISC_FEATURE - Xaa is F4OMe
  MOD_RES 14: note = METHYLATION
AVXVWNYXIIKRFYC

SEQ ID NO: 33 - protein, 15 aa, synthetic construct
  REGION 1..15: note = Synthesized polypeptide
  MOD_RES 3: note = METHYLATION
  SITE 12: note = MISC_FEATURE - Xaa is dr
  MOD_RES 14: note = METHYLATION
AVFVWNYYIIRXFYC

SEQ ID NO: 34 - protein, 15 aa, synthetic construct
  REGION 1..15: note = Synthesized polypeptide
  MOD_RES 3: note = METHYLATION
  SITE 8: note = MISC_FEATURE - Xaa is F4OMe
  SITE 12: note = MISC_FEATURE - Xaa is dr
  MOD_RES 14: note = METHYLATION
AVFVWNYXIIRXFYC

SEQ ID NO: 35 - protein, 15 aa, synthetic construct
  REGION 1..15: note = Synthesized polypeptide
  MOD_RES 3: note = METHYLATION
  MOD_RES 11: note = METHYLATION
  MOD_RES 14: note = METHYLATION
AVFVWNYYIIRRFYC

SEQ ID NO: 36 - protein, 15 aa, synthetic construct
  REGION 1..15: note = Synthesized polypeptide
  MOD_RES 3: note = METHYLATION
  SITE 8: note = MISC_FEATURE - Xaa is F4OMe
  MOD_RES 11: note = METHYLATION
  MOD_RES 14: note = METHYLATION
AVFVWNYXIIRRFYC

SEQ ID NO: 37 - protein, 15 aa, synthetic construct
  REGION 1..15: note = Synthesized polypeptide
  MOD_RES 3: note = METHYLATION
  SITE 5: note = MISC_FEATURE - Xaa is W5C
  SITE 8: note = MISC_FEATURE - Xaa is F4OMe
  MOD_RES 14: note = METHYLATION
AVFVXNYXIIRRYYC

SEQ ID NO: 38 - protein, 15 aa, synthetic construct
  REGION 1..15: note = Synthesized polypeptide
  SITE 3: note = MISC_FEATURE - Xaa is MeF3C
  SITE 8: note = MISC_FEATURE - Xaa is F4OMe
  MOD_RES 14: note = METHYLATION
AVXVWNYXIIRRYYC

SEQ ID NO: 39 - protein, 15 aa, synthetic construct
  REGION 1..15: note = Synthesized polypeptide
  SITE 3: note = MISC_FEATURE - Xaa is MeF3C
  SITE 5: note = MISC_FEATURE - Xaa is W1aa
  SITE 8: note = MISC_FEATURE - Xaa is F4OMe
  MOD_RES 14: note = METHYLATION
AVXVXNYXIERRFYC

SEQ ID NO: 40 - protein, 15 aa, synthetic construct
  REGION 1..15: note = Synthesized polypeptide
  SITE 3: note = MISC_FEATURE - Xaa is MeF3C
  SITE 5: note = MISC_FEATURE - Xaa is W1aa
  SITE 8: note = MISC_FEATURE - Xaa is F4aao
  MOD_RES 14: note = METHYLATION
AVXVXNYXIIRRFYC

SEQ ID NO: 41 - protein, 15 aa, synthetic construct
  REGION 1..15: note = Synthesized polypeptide
  MOD_RES 3: note = METHYLATION
  SITE 8: note = MISC_FEATURE - Xaa is F4aao
  MOD_RES 14: note = METHYLATION
AVFVWNYXIIRRYYC

SEQ ID NO: 42 - protein, 15 aa, synthetic construct
  REGION 1..15: note = Synthesized polypeptide
  MOD_RES 3: note = METHYLATION
  SITE 5: note = MISC_FEATURE - Xaa is W1aa
  SITE 8: note = MISC_FEATURE - Xaa is F4aao
  MOD_RES 14: note = METHYLATION
AVFVXNYXIIRRYYC

SEQ ID NO: 43 - protein, 15 aa, synthetic construct
  REGION 1..15: note = Synthesized polypeptide
  SITE 3: note = MISC_FEATURE - Xaa is MeF3C
  SITE 5: note = MISC_FEATURE - Xaa is W1aa
  SITE 8: note = MISC_FEATURE - Xaa is F4OMe
  MOD_RES 14: note = METHYLATION
AVXVXNYXIERRFYC

SEQ ID NO: 44 - protein, 15 aa, synthetic construct
  REGION 1..15: note = Synthesized polypeptide
  SITE 3: note = MISC_FEATURE - Xaa is MeF3C
  SITE 5: note = MISC_FEATURE - Xaa is W1aa
  SITE 8: note = MISC_FEATURE - Xaa is F4aao
  MOD_RES 14: note = METHYLATION
AVXVXNYXIIRRFYC

SEQ ID NO: 45 - protein, 15 aa, synthetic construct
  REGION 1..15: note = Synthesized polypeptide
  MOD_RES 3: note = METHYLATION
  SITE 8: note = MISC_FEATURE - Xaa is F4aao
  MOD_RES 14: note = METHYLATION
AVFVWNYXIIRRYYC

SEQ ID NO: 46 - protein, 15 aa, synthetic construct
  REGION 1..15: note = Synthesized polypeptide
  MOD_RES 3: note = METHYLATION
  SITE 5: note = MISC_FEATURE - Xaa is W1aa
  SITE 8: note = MISC_FEATURE - Xaa is F4aao
  MOD_RES 14: note = METHYLATION
AVFVXNYXIIRRYYC

SEQ ID NO: 47 - protein, 15 aa, synthetic construct
  REGION 1..15: note = Synthesized polypeptide
  SITE 3: note = MISC_FEATURE - Xaa is MeF3C
  SITE 5: note = MISC_FEATURE - Xaa is W1aa
  SITE 8: note = MISC_FEATURE - Xaa is F4aao
  MOD_RES 14: note = METHYLATION
AVXVXNYXIIRRFYC

SEQ ID NO: 48 - protein, 15 aa, synthetic construct
  REGION 1..15: note = Synthesized polypeptide
  SITE 3: note = MISC_FEATURE - Xaa is MeF3C
  SITE 5: note = MISC_FEATURE - Xaa is W1aa
  SITE 8: note = MISC_FEATURE - Xaa is 3Py
  SITE 13: note = MISC_FEATURE - Xaa is 4Py
  MOD_RES 14: note = METHYLATION
AVXVXNYXIIRRXYC

SEQ ID NO: 49 - protein, 15 aa, synthetic construct
  REGION 1..15: note = Synthesized polypeptide
  SITE 3: note = MISC_FEATURE - Xaa is MeF3C
  SITE 5: note = MISC_FEATURE - Xaa is W1aa
  SITE 7: note = MISC_FEATURE - Xaa is 3Py6NH2
  SITE 8: note = MISC_FEATURE - Xaa is 3Py
  SITE 13: note = MISC_FEATURE - Xaa is 4Py
  MOD_RES 14: note = METHYLATION
AVXVXNXXIIRRXYC

SEQ ID NO: 50 - protein, 15 aa, synthetic construct
  REGION 1..15: note = Synthesized polypeptide
  SITE 3: note = MISC_FEATURE - Xaa is MeF3C
  SITE 5: note = MISC_FEATURE - Xaa is W1aa
  SITE 7: note = MISC_FEATURE - Xaa is 3Py6NH2
  SITE 8: note = MISC_FEATURE - Xaa is F4OMe
  SITE 13: note = MISC_FEATURE - Xaa is 4Py
  MOD_RES 14: note = METHYLATION
AVXVXNXXIIRRXYC

SEQ ID NO: 51 - protein, 15 aa, synthetic construct
  REGION 1..15: note = Synthesized polypeptide
  SITE 3: note = MISC_FEATURE - Xaa is MeF3C
  SITE 8: note = MISC_FEATURE - Xaa is 3Py
  SITE 13: note = MISC_FEATURE - Xaa is 4Py
  MOD_RES 14: note = METHYLATION
AVXVWNYXIIRRXYC

SEQ ID NO: 52 - protein, 15 aa, synthetic construct
  REGION 1..15: note = Synthesized polypeptide
  SITE 3: note = MISC_FEATURE - Xaa is MeF3C
  SITE 7: note = MISC_FEATURE - Xaa is 3Py6NH2
  SITE 8: note = MISC_FEATURE - Xaa is 3Py
  SITE 13: note = MISC_FEATURE - Xaa is 4Py
  MOD_RES 14: note = METHYLATION
AVXVWNXXIIRRXYC

SEQ ID NO: 53 - protein, 15 aa, synthetic construct
  REGION 1..15: note = Synthesized polypeptide
  SITE 3: note = MISC_FEATURE - Xaa is MeF3C
  SITE 7: note = MISC_FEATURE - Xaa is 3Py6NH2
  SITE 8: note = MISC_FEATURE - Xaa is F4OMe
  SITE 13: note = MISC_FEATURE - Xaa is 4Py
  MOD_RES 14: note = METHYLATION
AVXVWNXXIIRRXYC

SEQ ID NO: 54 - protein, 15 aa, synthetic construct
  REGION 1..15: note = Synthesized polypeptide
  SITE 3: note = MISC_FEATURE - Xaa is MeF3C
  SITE 8: note = MISC_FEATURE - Xaa is 4Py
  SITE 13: note = MISC_FEATURE - Xaa is 4Py
  MOD_RES 14: note = METHYLATION
AVXVWNYXIIRRXYC

SEQ ID NO: 55 - protein, 15 aa, synthetic construct
  REGION 1..15: note = Synthesized polypeptide
  SITE 3: note = MISC_FEATURE - Xaa is Me3Py
  SITE 8: note = MISC_FEATURE - Xaa is F4OMe
  MOD_RES 14: note = METHYLATION
AVXVWNYXIIRRFYC

SEQ ID NO: 56 - protein, 15 aa, synthetic construct
  REGION 1..15: note = Synthesized polypeptide
  SITE 3: note = MISC_FEATURE - Xaa is Me4Py
  SITE 8: note = MISC_FEATURE - Xaa is F4OMe
  MOD_RES 14: note = METHYLATION
AVXVWNYXIIRRFYC

SEQ ID NO: 57 - protein, 15 aa, synthetic construct
  REGION 1..15: note = Synthesized polypeptide
  SITE 3: note = MISC_FEATURE - Xaa is MeF3C
  SITE 7: note = MISC_FEATURE - Xaa is 3Py6NH2
  SITE 8: note = MISC_FEATURE - Xaa is F4OMe
  MOD_RES 14: note = METHYLATION
AVXVWNXXIIRRFYC

SEQ ID NO: 58 - protein, 15 aa, synthetic construct
  REGION 1..15: note = Synthesized polypeptide
  SITE 3: note = MISC_FEATURE - Xaa is Me3Py
  SITE 8: note = MISC_FEATURE - Xaa is F4OMe
  SITE 13: note = MISC_FEATURE - Xaa is 4Py
  MOD_RES 14: note = METHYLATION
AVXVWNYXIIRRXYC

SEQ ID NO: 59 - protein, 15 aa, synthetic construct
  REGION 1..15: note = Synthesized polypeptide
  SITE 3: note = MISC_FEATURE - Xaa is MeF3C
  SITE 8: note = MISC_FEATURE - Xaa is F4OMe
  SITE 13: note = MISC_FEATURE - Xaa is 4Py
  MOD_RES 14: note = METHYLATION
AVXVWNYXIIRRXYC

SEQ ID NO: 60 - protein, 15 aa, synthetic construct
  REGION 1..15: note = Synthesized polypeptide
  SITE 3: note = MISC_FEATURE - Xaa is MeF3C
  SITE 8: note = MISC_FEATURE - Xaa is 3Py
  MOD_RES 14: note = METHYLATION
AVXVWNYXIIRRFYC

SEQ ID NO: 61 - protein, 15 aa, synthetic construct
  REGION 1..15: note = Synthesized polypeptide
  SITE 3: note = MISC_FEATURE - Xaa is MeF3C
  SITE 8: note = MISC_FEATURE - Xaa is 4Py
  MOD_RES 14: note = METHYLATION
AVXVWNYXIIRRFYC

SEQ ID NO: 62 - protein, 15 aa, synthetic construct
  REGION 1..15: note = Synthesized polypeptide
  SITE 3: note = MISC_FEATURE - Xaa is MeF3C
  SITE 7: note = MISC_FEATURE - Xaa is 3Py6NH2
  SITE 8: note = MISC_FEATURE - Xaa is 4Py
  SITE 13: note = MISC_FEATURE - Xaa is 4Py
  MOD_RES 14: note = METHYLATION
AVXVWNXXIIRRXYC

SEQ ID NO: 63 - protein, 15 aa, synthetic construct
  REGION 1..15: note = Synthesized polypeptide
  SITE 3: note = MISC_FEATURE - Xaa is Me3Py
  SITE 7: note = MISC_FEATURE - Xaa is 3Py6NH2
  SITE 8: note = MISC_FEATURE - Xaa is F4OMe
  MOD_RES 14: note = METHYLATION
AVXVWNXXIIRRFYC

SEQ ID NO: 64 - protein, 15 aa, synthetic construct
  REGION 1..15: note = Synthesized polypeptide
  SITE 3: note = MISC_FEATURE - Xaa is Me4Py
  SITE 7: note = MISC_FEATURE - Xaa is 3Py6NH2
  SITE 8: note = MISC_FEATURE - Xaa is F4OMe
  MOD_RES 14: note = METHYLATION
AVXVWNXXIIRRFYC

SEQ ID NO: 65 - protein, 15 aa, synthetic construct
  REGION 1..15: note = Synthesized polypeptide
  SITE 3: note = MISC_FEATURE - Xaa is MeF3C
  SITE 5: note = MISC_FEATURE - Xaa is W7N
  SITE 8: note = MISC_FEATURE - Xaa is F4OMe
  SITE 13: note = MISC_FEATURE - Xaa is 4Py
  MOD_RES 14: note = METHYLATION
AVXVXNYXIIRRXYC

SEQ ID NO: 66 - protein, 15 aa, synthetic construct
  REGION 1..15: note = Synthesized polypeptide
  SITE 3: note = MISC_FEATURE - Xaa is MeF3C
  SITE 8: note = MISC_FEATURE - Xaa is F4OMe
  SITE 13: note = MISC_FEATURE - Xaa is 4Py
  SITE 14: note = MISC_FEATURE - Xaa is Me3Py
AVXVWNYXIIRRXXC

SEQ ID NO: 67 - protein, 15 aa, synthetic construct
  REGION 1..15: note = Synthesized polypeptide
  SITE 3: note = MISC_FEATURE - Xaa is MeF3C
  SITE 8: note = MISC_FEATURE - Xaa is 3Py
  SITE 13: note = MISC_FEATURE - Xaa is 4Py
  MOD_RES 14: note = METHYLATION
AVXVWNYXIIQQXYC

SEQ ID NO: 68 - protein, 15 aa, synthetic construct
  REGION 1..15: note = Synthesized polypeptide
  SITE 3: note = MISC_FEATURE - Xaa is MeF3C
  SITE 8: note = MISC_FEATURE - Xaa is 3Py
  SITE 13: note = MISC_FEATURE - Xaa is 4Py
  MOD_RES 14: note = METHYLATION
AVXVWNYXIIRRXYC

SEQ ID NO: 69 - protein, 15 aa, synthetic construct
  REGION 1..15: note = Synthesized polypeptide
  SITE 3: note = MISC_FEATURE - Xaa is MeF3C
  SITE 8: note = MISC_FEATURE - Xaa is 3Py
  SITE 13: note = MISC_FEATURE - Xaa is 4Py
  MOD_RES 14: note = METHYLATION
AVXVWNYXIIRRXYC

SEQ ID NO: 70 - protein, 15 aa, synthetic construct
  REGION 1..15: note = Synthesized polypeptide
  SITE 3: note = MISC_FEATURE - Xaa is MeF3C
  SITE 5: note = MISC_FEATURE - Xaa is W1aa
  SITE 8: note = MISC_FEATURE - Xaa is F4OMe
  BINDING 12: note = PEG8Me
  MOD_RES 14: note = METHYLATION
AVXVXNYXIIREFYC

SEQ ID NO: 71 - protein, 15 aa, synthetic construct
  REGION 1..15: note = Synthesized polypeptide
  SITE 3: note = MISC_FEATURE - Xaa is MeF3C
  SITE 5: note = MISC_FEATURE - Xaa is W1aa
  SITE 7: note = MISC_FEATURE - Xaa is 3Py6NH2
  SITE 8: note = MISC_FEATURE - Xaa is F4aao
  MOD_RES 14: note = METHYLATION
AVXVXNXXIIRRFYC

SEQ ID NO: 72 - protein, 15 aa, synthetic construct
  REGION 1..15: note = Synthesized polypeptide
  SITE 3: note = MISC_FEATURE - Xaa is MeF3C
  SITE 5: note = MISC_FEATURE - Xaa is W1aa
  SITE 7: note = MISC_FEATURE - Xaa is 3Py6NH2
  SITE 8: note = MISC_FEATURE - Xaa is F4OMe
  SITE 13: note = MISC_FEATURE - Xaa is F3COO
  MOD_RES 14: note = METHYLATION
AVXVXNXXIIRRXYC

SEQ ID NO: 73 - protein, 15 aa, synthetic construct
  REGION 1..15: note = Synthesized polypeptide
  SITE 3: note = MISC_FEATURE - Xaa is MeF3C
  SITE 5: note = MISC_FEATURE - Xaa is W1aa
  SITE 8: note = MISC_FEATURE - Xaa is 3Py
  BINDING 12: note = PEG8Me
  MOD_RES 14: note = METHYLATION
AVXVXNYXIIREFYC

SEQ ID NO: 74 - protein, 15 aa, synthetic construct
  REGION 1..15: note = Synthesized polypeptide
  SITE 3: note = MISC_FEATURE - Xaa is MeF3C
  SITE 5: note = MISC_FEATURE - Xaa is W1aa
  SITE 8: note = MISC_FEATURE - Xaa is 3Py
  SITE 13: note = MISC_FEATURE - Xaa is F3COO
  MOD_RES 14: note = METHYLATION
AVXVXNYXIIRRXYC

SEQ ID NO: 75 - protein, 15 aa, synthetic construct
  REGION 1..15: note = Synthesized polypeptide
  SITE 3: note = MISC_FEATURE - Xaa is MeF3C
  SITE 5: note = MISC_FEATURE - Xaa is W1aa
  SITE 8: note = MISC_FEATURE - Xaa is F4aao
  SITE 13: note = MISC_FEATURE - Xaa is F3COO
  MOD_RES 14: note = METHYLATION
AVXVXNYXIIRRXYC

SEQ ID NO: 76 - protein, 15 aa, synthetic construct
  REGION 1..15: note = Synthesized polypeptide
  SITE 3: note = MISC_FEATURE - Xaa is MeF3C
  SITE 5: note = MISC_FEATURE - Xaa is W1aa
  SITE 8: note = MISC_FEATURE - Xaa is F4aao
  SITE 13: note = MISC_FEATURE - Xaa is 4Py
  MOD_RES 14: note = METHYLATION
AVXVXNYXIIRRXYC

SEQ ID NO: 77 - protein, 15 aa, synthetic construct
  REGION 1..15: note = Synthesized polypeptide
  SITE 3: note = MISC_FEATURE - Xaa is MeF3C
  SITE 5: note = MISC_FEATURE - Xaa is W1aa
  SITE 8: note = MISC_FEATURE - Xaa is F4OMe
  BINDING 12: note = PEG8Me
  SITE 13: note = MISC_FEATURE - Xaa is F3COO
  MOD_RES 14: note = METHYLATION
AVXVXNYXIIREXYC

SEQ ID NO: 78 - protein, 15 aa, synthetic construct
  REGION 1..15: note = Synthesized polypeptide
  SITE 3: note = MISC_FEATURE - Xaa is MeF3C
  SITE 5: note = MISC_FEATURE - Xaa is W1aa
  SITE 8: note = MISC_FEATURE - Xaa is F4OMe
  BINDING 12: note = PEG8Me
  SITE 13: note = MISC_FEATURE - Xaa is 4Py
  MOD_RES 14: note = METHYLATION
AVXVXNYXIIREXYC

SEQ ID NO: 79 - protein, 15 aa, synthetic construct
  REGION 1..15: note = Synthesized polypeptide
  SITE 3: note = MISC_FEATURE - Xaa is MeF3C
  SITE 5: note = MISC_FEATURE - Xaa is W1aa
  SITE 7: note = MISC_FEATURE - Xaa is 3Py6NH2
  SITE 8: note = MISC_FEATURE - Xaa is 3Py
  SITE 13: note = MISC_FEATURE - Xaa is F3COO
  MOD_RES 14: note = METHYLATION
AVXVXNXXIIRRXYC

SEQ ID NO: 80 - protein, 15 aa, synthetic construct
  REGION 1..15: note = Synthesized polypeptide
  SITE 3: note = MISC_FEATURE - Xaa is MeF3C
  SITE 5: note = MISC_FEATURE - Xaa is W1aa
  SITE 7: note = MISC_FEATURE - Xaa is 3Py6NH2
  SITE 8: note = MISC_FEATURE - Xaa is F4aao
  SITE 13: note = MISC_FEATURE - Xaa is 4Py
  MOD_RES 14: note = METHYLATION
AVXVXNXXIIRRXYC

SEQ ID NO: 81 - protein, 15 aa, synthetic construct
  REGION 1..15: note = Synthesized polypeptide
  SITE 3: note = MISC_FEATURE - Xaa is MeF3C
  SITE 5: note = MISC_FEATURE - Xaa is W1aa
  SITE 7: note = MISC_FEATURE - Xaa is 3Py6NH2
  SITE 8: note = MISC_FEATURE - Xaa is F4aao
  SITE 13: note = MISC_FEATURE - Xaa is F3COO
  MOD_RES 14: note = METHYLATION
AVXVXNXXIIRRXYC

SEQ ID NO: 82 - protein, 15 aa, synthetic construct
  REGION 1..15: note = Synthesized polypeptide
  SITE 3: note = MISC_FEATURE - Xaa is MeF3C
  SITE 5: note = MISC_FEATURE - Xaa is W1aa
  SITE 8: note = MISC_FEATURE - Xaa is F4aao
  BINDING 12: note = PEG8Me
  SITE 13: note = MISC_FEATURE - Xaa is 4Py
  MOD_RES 14: note = METHYLATION
AVXVXNYXIIREXYC

SEQ ID NO: 83 - protein, 15 aa, synthetic construct
  REGION 1..15: note = Synthesized polypeptide
  SITE 3: note = MISC_FEATURE - Xaa is MeF3C
  SITE 5: note = MISC_FEATURE - Xaa is W1aa
  SITE 8: note = MISC_FEATURE - Xaa is 3Py
  BINDING 12: note = PEG8Me
  SITE 13: note = MISC_FEATURE - Xaa is 4Py
  MOD_RES 14: note = METHYLATION
AVXVXNYXIIREXYC

SEQ ID NO: 84 - protein, 15 aa, synthetic construct
  REGION 1..15: note = Synthesized polypeptide
  SITE 3: note = MISC_FEATURE - Xaa is MeF3C
  SITE 5: note = MISC_FEATURE - Xaa is W1aa
  SITE 8: note = MISC_FEATURE - Xaa is 3Py
  BINDING 12: note = PEG8Me
  SITE 13: note = MISC_FEATURE - Xaa is F3COO
  MOD_RES 14: note = METHYLATION
AVXVXNYXIIREXYC

SEQ ID NO: 85 - protein, 15 aa, synthetic construct
  REGION 1..15: note = Synthesized polypeptide
  SITE 3: note = MISC_FEATURE - Xaa is MeF3C
  SITE 5: note = MISC_FEATURE - Xaa is W1aa
  SITE 7: note = MISC_FEATURE - Xaa is 3Py6NH2
  SITE 8: note = MISC_FEATURE - Xaa is 3Py
  BINDING 12: note = PEG8Me
  SITE 13: note = MISC_FEATURE - Xaa is F3COO
  MOD_RES 14: note = METHYLATION
AVXVXNXXIIREXYC

SEQ ID NO: 86 - protein, 15 aa, synthetic construct
  REGION 1..15: note = Synthesized polypeptide
  SITE 3: note = MISC_FEATURE - Xaa is MeF3C
  SITE 5: note = MISC_FEATURE - Xaa is W1aa
  SITE 7: note = MISC_FEATURE - Xaa is 3Py6NH2
  SITE 8: note = MISC_FEATURE - Xaa is 3Py
  BINDING 12: note = PEG8Me
  SITE 13: note = MISC_FEATURE - Xaa is 4Py
  MOD_RES 14: note = METHYLATION
AVXVXNXXIIREXYC

SEQ ID NO: 87 - protein, 15 aa, synthetic construct
  REGION 1..15: note = Synthesized polypeptide
  SITE 3: note = MISC_FEATURE - Xaa is MeF3C
  SITE 5: note = MISC_FEATURE - Xaa is W1aa
  SITE 7: note = MISC_FEATURE - Xaa is 3Py6NH2
  SITE 8: note = MISC_FEATURE - Xaa is F4aao
  BINDING 12: note = PEG8Me
  SITE 13: note = MISC_FEATURE - Xaa is F3COO
  MOD_RES 14: note = METHYLATION
AVXVXNXXIIREXYC

SEQ ID NO: 88 - protein, 15 aa, synthetic construct
  REGION 1..15: note = Synthesized polypeptide
  SITE 3: note = MISC_FEATURE - Xaa is MeF3C
  SITE 5: note = MISC_FEATURE - Xaa is W1aa
  SITE 7: note = MISC_FEATURE - Xaa is 3Py6NH2
  SITE 8: note = MISC_FEATURE - Xaa is F4aao
  BINDING 12: note = PEG8Me
  SITE 13: note = MISC_FEATURE - Xaa is 4Py
  MOD_RES 14: note = METHYLATION
AVXVXNXXIIREXYC

SEQ ID NO: 89 - protein, 15 aa, synthetic construct
  REGION 1..15: note = Synthesized polypeptide
  SITE 3: note = MISC_FEATURE - Xaa is MeF3C
  SITE 8: note = MISC_FEATURE - Xaa is F4aao
  BINDING 12: note = PEG8Me
  MOD_RES 14: note = METHYLATION
AVXVWNYXIIREFYC

SEQ ID NO: 90 - protein, 15 aa, synthetic construct
  REGION 1..15: note = Synthesized polypeptide
  SITE 3: note = MISC_FEATURE - Xaa is MeF3C
  SITE 8: note = MISC_FEATURE - Xaa is F4OMe
  BINDING 12: note = PEG8Me
  SITE 13: note = MISC_FEATURE - Xaa is F3COO
  MOD_RES 14: note = METHYLATION
AVXVWNYXIIREXYC

SEQ ID NO: 91 - protein, 15 aa, synthetic construct
  REGION 1..15: note = Synthesized polypeptide
  SITE 3: note = MISC_FEATURE - Xaa is MeF3C
  SITE 7: note = MISC_FEATURE - Xaa is 3Py6NH2
  SITE 8: note = MISC_FEATURE - Xaa is F4aao
  SITE 13: note = MISC_FEATURE - Xaa is F3COO
  MOD_RES 14: note = METHYLATION
AVXVWNXXIIRRXYC

SEQ ID NO: 92 - protein, 15 aa, synthetic construct
  REGION 1..15: note = Synthesized polypeptide
  SITE 3: note = MISC_FEATURE - Xaa is MeF3C
  SITE 7: note = MISC_FEATURE - Xaa is 3Py6NH2
  SITE 8: note = MISC_FEATURE - Xaa is F4aao
  SITE 13: note = MISC_FEATURE - Xaa is 4Py
  MOD_RES 14: note = METHYLATION
AVXVWNXXIIRRXYC

SEQ ID NO: 93 - protein, 15 aa, synthetic construct
  REGION 1..15: note = Synthesized polypeptide
  SITE 3: note = MISC_FEATURE - Xaa is MeF3C
  SITE 8: note = MISC_FEATURE - Xaa is 3Py
  BINDING 12: note = PEG8Me
  SITE 13: note = MISC_FEATURE - Xaa is F3COO
  MOD_RES 14: note = METHYLATION
AVXVWNYXIIREXYC

SEQ ID NO: 94 - protein, 15 aa, synthetic construct
  REGION 1..15: note = Synthesized polypeptide
  SITE 3: note = MISC_FEATURE - Xaa is MeF3C
  SITE 8: note = MISC_FEATURE - Xaa is 3Py
  BINDING 12: note = PEG8Me
  SITE 13: note = MISC_FEATURE - Xaa is 4Py
  MOD_RES 14: note = METHYLATION
AVXVWNYXIIREXYC

SEQ ID NO: 95 - protein, 15 aa, synthetic construct
  REGION 1..15: note = Synthesized polypeptide
  SITE 3: note = MISC_FEATURE - Xaa is MeF3C
  SITE 8: note = MISC_FEATURE - Xaa is F4aao
  BINDING 12: note = PEG8Me
  SITE 13: note = MISC_FEATURE - Xaa is F3COO
  MOD_RES 14: note = METHYLATION
AVXVWNYXIIREXYC

SEQ ID NO: 96 - protein, 15 aa, synthetic construct
  REGION 1..15: note = Synthesized polypeptide
  SITE 3: note = MISC_FEATURE - Xaa is MeF3C
  SITE 8: note = MISC_FEATURE - Xaa is F4aao
  BINDING 12: note = PEG8Me
  SITE 13: note = MISC_FEATURE - Xaa is 4Py
  MOD_RES 14: note = METHYLATION
AVXVWNYXIIREXYC

SEQ ID NO: 97 - protein, 15 aa, synthetic construct
  REGION 1..15: note = Synthesized polypeptide
  SITE 3: note = MISC_FEATURE - Xaa is MeF3C
  SITE 7: note = MISC_FEATURE - Xaa is 3Py6NH2
  SITE 8: note = MISC_FEATURE - Xaa is 3Py
  BINDING 12: note = PEG8Me
  SITE 13: note = MISC_FEATURE - Xaa is F3COO
  MOD_RES 14: note = METHYLATION
AVXVWNXXIIREXYC

SEQ ID NO: 98 - protein, 15 aa, synthetic construct
  REGION 1..15: note = Synthesized polypeptide
  SITE 3: note = MISC_FEATURE - Xaa is MeF3C
  SITE 7: note = MISC_FEATURE - Xaa is 3Py6NH2
  SITE 8: note = MISC_FEATURE - Xaa is 3Py
  BINDING 12: note = PEG8Me
  SITE 13: note = MISC_FEATURE - Xaa is 4Py
  MOD_RES 14: note = METHYLATION
AVXVWNXXIIREXYC

SEQ ID NO: 99 - protein, 15 aa, synthetic construct
  REGION 1..15: note = Synthesized polypeptide
  SITE 3: note = MISC_FEATURE - Xaa is MeF3C
  SITE 7: note = MISC_FEATURE - Xaa is 3Py6NH2
  SITE 8: note = MISC_FEATURE - Xaa is F4aao
  BINDING 12: note = PEG8Me
  SITE 13: note = MISC_FEATURE - Xaa is F3COO
  MOD_RES 14: note = METHYLATION
AVXVWNXXIIREXYC

SEQ ID NO: 100 - protein, 15 aa, synthetic construct
  REGION 1..15: note = Synthesized polypeptide
  SITE 3: note = MISC_FEATURE - Xaa is MeF3C
  SITE 7: note = MISC_FEATURE - Xaa is 3Py6NH2
  SITE 8: note = MISC_FEATURE - Xaa is F4aao
  BINDING 12: note = PEG8Me
  SITE 13: note = MISC_FEATURE - Xaa is 4Py
  MOD_RES 14: note = METHYLATION
AVXVWNXXIIREXYC

SEQ ID NO: 101 - protein, 15 aa, synthetic construct
  REGION 1..15: note = Synthesized polypeptide
  SITE 3: note = MISC_FEATURE - Xaa is MeF3C
  SITE 5: note = MISC_FEATURE - Xaa is W1aa
  SITE 8: note = MISC_FEATURE - Xaa is F4aao
  BINDING 11: note = PEG8Me
  MOD_RES 14: note = METHYLATION
AVXVXNYXIIERFYC

SEQ ID NO: 102 - protein, 15 aa, synthetic construct
  REGION 1..15: note = Synthesized polypeptide
  SITE 3: note = MISC_FEATURE - Xaa is MeF3C
  SITE 5: note = MISC_FEATURE - Xaa is W1aa
  SITE 8: note = MISC_FEATURE - Xaa is F4aao
  BINDING 12: note = PEG8Me
  MOD_RES 14: note = METHYLATION
AVXVXNYXIIREFYC

SEQ ID NO: 103 - protein, 15 aa, synthetic construct
  REGION 1..15: note = Synthesized polypeptide
  SITE 3: note = MISC_FEATURE - Xaa is MeF3C
  SITE 5: note = MISC_FEATURE - Xaa is W1aa
  SITE 8: note = MISC_FEATURE - Xaa is F4aao
  BINDING 11: note = PEG8Me
  SITE 13: note = MISC_FEATURE - Xaa is F3COO
  MOD_RES 14: note = METHYLATION
AVXVXNYXIIERXYC

SEQ ID NO: 104 - protein, 15 aa, synthetic construct
  REGION 1..15: note = Synthesized polypeptide
  SITE 3: note = MISC_FEATURE - Xaa is MeF3C
  SITE 5: note = MISC_FEATURE - Xaa is W1aa
  SITE 8: note = MISC_FEATURE - Xaa is F4aao
  MOD_RES 14: note = METHYLATION
AVXVXNYXIIQRFYC

SEQ ID NO: 105 - protein, 15 aa, synthetic construct
  REGION 1..15: note = Synthesized polypeptide
  SITE 3: note = MISC_FEATURE - Xaa is MeF3C
  SITE 5: note = MISC_FEATURE - Xaa is W1aa
  SITE 8: note = MISC_FEATURE - Xaa is F4aao
  MOD_RES 14: note = METHYLATION
AVXVXNYXIIRQFYC

SEQ ID NO: 106 - protein, 15 aa, synthetic construct
  REGION 1..15: note = Synthesized polypeptide
  MOD_RES 3: note = METHYLATION
  MOD_RES 14: note = METHYLATION
AVFVWNYYIIRRYYC

SEQ ID NO: 107 - protein, 15 aa, synthetic construct
  REGION 1..15: note = Synthesized polypeptide
  MOD_RES 3: note = METHYLATION
  MOD_RES 14: note = METHYLATION
AVFVWNYYIIRRYYC

SEQ ID NO: 108 - protein, 15 aa, synthetic construct
  REGION 1..15: note = Synthesized polypeptide
  SITE 3: note = MISC_FEATURE - Xaa is MeF3C
  SITE 5: note = MISC_FEATURE - Xaa is W1aa
  SITE 8: note = MISC_FEATURE - Xaa is F4OMe
  MOD_RES 14: note = METHYLATION
AVXVXNYXIIRRFYC

SEQ ID NO: 109 - protein, 15 aa, synthetic construct
  REGION 1..15: note = Synthesized polypeptide
  SITE 3: note = MISC_FEATURE - Xaa is MeF3C
  SITE 8: note = MISC_FEATURE - Xaa is F4aao
  MOD_RES 14: note = METHYLATION
AVXVWNYXIIRRFYC

SEQ ID NO: 110 - protein, 15 aa, synthetic construct
  REGION 1..15: note = Synthesized polypeptide
  SITE 3: note = MISC_FEATURE - Xaa is MeF3C
  SITE 5: note = MISC_FEATURE - Xaa is W1aa
  SITE 8: note = MISC_FEATURE - Xaa is F4aao
  BINDING 11: note = PEG4Me
  MOD_RES 14: note = METHYLATION
AVXVXNYXIIERFYC

SEQ ID NO: 111 - protein, 15 aa, synthetic construct
  REGION 1..15: note = Synthesized polypeptide
  SITE 3: note = MISC_FEATURE - Xaa is MeF3C
  SITE 5: note = MISC_FEATURE - Xaa is W1aa
  SITE 8: note = MISC_FEATURE - Xaa is F4aao
  BINDING 11: note = NHdPEG1Me
  MOD_RES 14: note = METHYLATION
AVXVXNYXIIERFYC

SEQ ID NO: 112 - protein, 15 aa, synthetic construct
  REGION 1..15: note = Synthesized polypeptide
  SITE 3: note = MISC_FEATURE - Xaa is MeF3C
  SITE 8: note = MISC_FEATURE - Xaa is F4aao
  BINDING 11: note = PEG8Me
  MOD_RES 14: note = METHYLATION
AVXVWNYXIIERFYC

SEQ ID NO: 113 - protein, 15 aa, synthetic construct
  REGION 1..15: note = Synthesized polypeptide
  SITE 3: note = MISC_FEATURE - Xaa is MeF3C
  SITE 8: note = MISC_FEATURE - Xaa is F4aao
  BINDING 11: note = PEG4Me
  MOD_RES 14: note = METHYLATION
AVXVWNYXIIERFYC

SEQ ID NO: 114 - protein, 15 aa, synthetic construct
  REGION 1..15: note = Synthesized polypeptide
  SITE 3: note = MISC_FEATURE - Xaa is MeF3C
  SITE 8: note = MISC_FEATURE - Xaa is F4aao
  BINDING 11: note = NHdPEG1Me
  SITE 13: note = MISC_FEATURE - Xaa is F3COO
  MOD_RES 14: note = METHYLATION
AVXVWNYXIIERXYC

SEQ ID NO: 115 - protein, 15 aa, synthetic construct
  REGION 1..15: note = Synthesized polypeptide
  SITE 3: note = MISC_FEATURE - Xaa is MeF3C
  SITE 5: note = MISC_FEATURE - Xaa is W1aa
  SITE 8: note = MISC_FEATURE - Xaa is F4aao
  BINDING 11: note = PEG4Me
  SITE 12: note = MISC_FEATURE - Xaa is KCOpipzaa
  MOD_RES 14: note = METHYLATION
AVXVXNYXIIEXFYC

SEQ ID NO: 116 - protein, 15 aa, synthetic construct
  REGION 1..15: note = Synthesized polypeptide
  SITE 3: note = MISC_FEATURE - Xaa is MeF3C
  SITE 8: note = MISC_FEATURE - Xaa is F4aao
  BINDING 11: note = PEG4Me
  SITE 12: note = MISC_FEATURE - Xaa is KCOpipzaa
  MOD_RES 14: note = METHYLATION
AVXVWNYXIIEXFYC

SEQ ID NO: 117 - protein, 15 aa, synthetic construct
  REGION 1..15: note = Synthesized polypeptide
  SITE 3: note = MISC_FEATURE - Xaa is MeF3C
  SITE 5: note = MISC_FEATURE - Xaa is W1aa
  SITE 7: note = MISC_FEATURE - Xaa is 3Py6NH2
  SITE 8: note = MISC_FEATURE - Xaa is F4aao
  BINDING 11: note = PEG4Me
  SITE 13: note = MISC_FEATURE - Xaa is 4Py
  MOD_RES 14: note = METHYLATION
AVXVXNXXIIERXYC

SEQ ID NO: 118 - protein, 15 aa, synthetic construct
  REGION 1..15: note = Synthesized polypeptide
  SITE 3: note = MISC_FEATURE - Xaa is MeF3C
  SITE 7: note = MISC_FEATURE - Xaa is 3Py6NH2
  SITE 8: note = MISC_FEATURE - Xaa is F4aao
  BINDING 11: note = PEG4Me
  SITE 12: note = MISC_FEATURE - Xaa is KCOpipzaa
  SITE 13: note = MISC_FEATURE - Xaa is 4Py
  MOD_RES 14: note = METHYLATION
AVXVWNXXIIEXXYC

SEQ ID NO: 119 - protein, 15 aa, synthetic construct
  REGION 1..15: note = Synthesized polypeptide
  SITE 3: note = MISC_FEATURE - Xaa is MeF3C
  SITE 5: note = MISC_FEATURE - Xaa is W1aa
  SITE 8: note = MISC_FEATURE - Xaa is F4aao
  BINDING 11: note = PEG4Me
  SITE 12: note = MISC_FEATURE - Xaa is Kmor
  MOD_RES 14: note = METHYLATION
AVXVXNYXIIEXFYC

SEQ ID NO: 120 - protein, 15 aa, synthetic construct
  REGION 1..15: note = Synthesized polypeptide
  SITE 3: note = MISC_FEATURE - Xaa is MeF3C
  SITE 8: note = MISC_FEATURE - Xaa is F4aao
  BINDING 11: note = PEG4Me
  SITE 12: note = MISC_FEATURE - Xaa is Kmor
  MOD_RES 14: note = METHYLATION
AVXVWNYXIIEXFYC

SEQ ID NO: 121 - protein, 15 aa, synthetic construct
  REGION 1..15: note = Synthesized polypeptide
  SITE 3: note = MISC_FEATURE - Xaa is MeF3C
  SITE 8: note = MISC_FEATURE - Xaa is F4aao
  BINDING 11: note = PEG4Me
  MOD_RES 14: note = METHYLATION
AVXVWNYXIIEKFYC

SEQ ID NO: 122 - protein, 15 aa, synthetic construct
  REGION 1..15: note = Synthesized polypeptide
  SITE 3: note = MISC_FEATURE - Xaa is MeF3C
  SITE 8: note = MISC_FEATURE - Xaa is F4aao
  BINDING 11: note = PEG4Me
  SITE 12: note = MISC_FEATURE - Xaa is KdMe
  MOD_RES 14: note = METHYLATION
AVXVWNYXIIEXFYC

SEQ ID NO: 123 - protein, 15 aa, synthetic construct
  REGION 1..15: note = Synthesized polypeptide
  SITE 3: note = MISC_FEATURE - Xaa is MeF3C
  SITE 8: note = MISC_FEATURE - Xaa is F4aao
  BINDING 11: note = PEG4Me
  MOD_RES 14: note = METHYLATION
AVXVWNYXIIEQFYC

SEQ ID NO: 124 - protein, 15 aa, synthetic construct
  REGION 1..15: note = Synthesized polypeptide
  SITE 3: note = MISC_FEATURE - Xaa is MeF3C
  SITE 8: note = MISC_FEATURE - Xaa is F4aao
  BINDING 11: note = PEG4Me
  BINDING 13: note = PEG4Me
  MOD_RES 14: note = METHYLATION
AVXVWNYXIIEREYC

SEQ ID NO: 125 - protein, 15 aa, synthetic construct
  REGION 1..15: note = Synthesized polypeptide
  SITE 3: note = MISC_FEATURE - Xaa is MeF3C
  SITE 8: note = MISC_FEATURE - Xaa is F4aao
  BINDING 11: note = PEG4Me
  BINDING 13: note = PEG4Me
  MOD_RES 14: note = METHYLATION
AVXVWNYXIIEREYC

SEQ ID NO: 126 - protein, 15 aa, synthetic construct
  REGION 1..15: note = Synthesized polypeptide
  SITE 3: note = MISC_FEATURE - Xaa is MeF3C
  SITE 8: note = MISC_FEATURE - Xaa is F4aao
  BINDING 11: note = PEG4Me
  SITE 13: note = MISC_FEATURE - Xaa is F3COO(PEG4Me)
  MOD_RES 14: note = METHYLATION
AVXVWNYXIIERXYC

SEQ ID NO: 127 - protein, 15 aa, synthetic construct
  REGION 1..15: note = Synthesized polypeptide
  SITE 3: note = MISC_FEATURE - Xaa is MeF3C
  SITE 8: note = MISC_FEATURE - Xaa is F4aao
  SITE 13: note = MISC_FEATURE - Xaa is F3COO(PEG4Me)
  SITE 14: note = MISC_FEATURE - Xaa is MeF4COO(PEG4Me)
AVXVWNYXIIQRXXC

SEQ ID NO: 128 - protein, 15 aa, synthetic construct
  REGION 1..15: note = Synthesized polypeptide
  SITE 3: note = MISC_FEATURE - Xaa is MeF3C
  SITE 8: note = MISC_FEATURE - Xaa is F4aao
  SITE 13: note = MISC_FEATURE - Xaa is F3COO(PEG4Me)
  SITE 14: note = MISC_FEATURE - Xaa is MeF3COO(PEG4Me)
AVXVWNYXIIQRXXC

SEQ ID NO: 129 - protein, 15 aa, synthetic construct
  REGION 1..15: note = Synthesized polypeptide
  SITE 3: note = MISC_FEATURE - Xaa is MeF3C
  SITE 8: note = MISC_FEATURE - Xaa is F4aao
  SITE 13: note = MISC_FEATURE - Xaa is F3COO(PEG4Me)
  SITE 14: note = MISC_FEATURE - Xaa is MeF3COO(PEG4Me)
AVXVWNYXIIQRXXC

SEQ ID NO: 130 - protein, 15 aa, synthetic construct
  REGION 1..15: note = Synthesized polypeptide
  SITE 3: note = MISC_FEATURE - Xaa is MeF3C
  SITE 5: note = MISC_FEATURE - Xaa is W7N
  SITE 8: note = MISC_FEATURE - Xaa is F4aao
  BINDING 11: note = PEG4Me
  SITE 13: note = MISC_FEATURE - Xaa is F3COO(PEG4Me)
  MOD_RES 14: note = METHYLATION
AVXVXNYXIIERXYC

SEQ ID NO: 131 - protein, 15 aa, synthetic construct
  REGION 1..15: note = Synthesized polypeptide
  SITE 3: note = MISC_FEATURE - Xaa is MeF3C
  SITE 5: note = MISC_FEATURE - Xaa is W7N
  SITE 8: note = MISC_FEATURE - Xaa is F4aao
  SITE 13: note = MISC_FEATURE - Xaa is F3COO(PEG4Me)
  SITE 14: note = MISC_FEATURE - Xaa is MeF4COO(PEG4Me)
AVXVXNYXIIQRXXC

SEQ ID NO: 132 - protein, 15 aa, synthetic construct
  REGION 1..15: note = Synthesized polypeptide
  SITE 3: note = MISC_FEATURE - Xaa is MeF3C
  SITE 5: note = MISC_FEATURE - Xaa is W7N
  SITE 8: note = MISC_FEATURE - Xaa is F4aao
  SITE 13: note = MISC_FEATURE - Xaa is F3COO(PEG4Me)
  SITE 14: note = MISC_FEATURE - Xaa is MeF3COO(PEG4Me)
AVXVXNYXIIQRXXC

SEQ ID NO: 133 - protein, 15 aa, synthetic construct
  REGION 1..15: note = Synthesized polypeptide
  SITE 3: note = MISC_FEATURE - Xaa is MeF3C
  SITE 5: note = MISC_FEATURE - Xaa is W7N
  SITE 8: note = MISC_FEATURE - Xaa is F4aao
  BINDING 11: note = PEG4Me
  MOD_RES 14: note = METHYLATION
AVXVXNYXIIERFYC

SEQ ID NO: 134 - protein, 15 aa, synthetic construct
  REGION 1..15: note = Synthesized polypeptide
  SITE 3: note = MISC_FEATURE - Xaa is MeF3C
  SITE 5: note = MISC_FEATURE - Xaa is W1aa
  SITE 8: note = MISC_FEATURE - Xaa is F4aao
  SITE 13: note = MISC_FEATURE - Xaa is 4Py
  MOD_RES 14: note = METHYLATION
AVXVXNYXIIQRXYC

SEQ ID NO: 135 - protein, 15 aa, synthetic construct
  REGION 1..15: note = Synthesized polypeptide
  SITE 3: note = MISC_FEATURE - Xaa is MeF3C
  SITE 5: note = MISC_FEATURE - Xaa is W1aa
  SITE 8: note = MISC_FEATURE - Xaa is F4aao
  SITE 12: note = MISC_FEATURE - Xaa is Kmor
  SITE 13: note = MISC_FEATURE - Xaa is 4Py
  MOD_RES 14: note = METHYLATION
AVXVXNYXIIQXXYC

SEQ ID NO: 136 - protein, 15 aa, synthetic construct
  REGION 1..15: note = Synthesized polypeptide
  SITE 3: note = MISC_FEATURE - Xaa is MeF3C
  SITE 5: note = MISC_FEATURE - Xaa is W1aa
  SITE 8: note = MISC_FEATURE - Xaa is F4aao
  SITE 13: note = MISC_FEATURE - Xaa is F3COO
  MOD_RES 14: note = METHYLATION
AVXVXNYXIIQRXYC

SEQ ID NO: 137 - protein, 15 aa, synthetic construct
  REGION 1..15: note = Synthesized polypeptide
  SITE 3: note = MISC_FEATURE - Xaa is MeF3C
  SITE 5: note = MISC_FEATURE - Xaa is W7N
  SITE 8: note = MISC_FEATURE - Xaa is F4aao
  SITE 13: note = MISC_FEATURE - Xaa is 4Py
  MOD_RES 14: note = METHYLATION
AVXVXNYXIIQRXYC

SEQ ID NO: 138 - protein, 15 aa, synthetic construct
  REGION 1..15: note = Synthesized polypeptide
  SITE 3: note = MISC_FEATURE - Xaa is MeF3C
  SITE 5: note = MISC_FEATURE - Xaa is W7N
  SITE 8: note = MISC_FEATURE - Xaa is F4aao
  SITE 12: note = MISC_FEATURE - Xaa is Kmor
  SITE 13: note = MISC_FEATURE - Xaa is 4Py
  MOD_RES 14: note = METHYLATION
AVXVXNYXIIQXXYC

SEQ ID NO: 139 - protein, 15 aa, synthetic construct
  REGION 1..15: note = Synthesized polypeptide
  SITE 3: note = MISC_FEATURE - Xaa is MeF3C
  SITE 5: note = MISC_FEATURE - Xaa is W7N
  SITE 8: note = MISC_FEATURE - Xaa is F4aao
  BINDING 11: note = PEG8Me
  SITE 12: note = MISC_FEATURE - Xaa is Kmor
  SITE 13: note = MISC_FEATURE - Xaa is 4Py
  MOD_RES 14: note = METHYLATION
AVXVXNYXIIEXXYC

SEQ ID NO: 140 - protein, 15 aa, synthetic construct
  REGION 1..15: note = Synthesized polypeptide
  SITE 3: note = MISC_FEATURE - Xaa is MeF3C
  SITE 5: note = MISC_FEATURE - Xaa is W7N
  SITE 8: note = MISC_FEATURE - Xaa is F4aao
  SITE 12: note = MISC_FEATURE - Xaa is Kmor
  SITE 13: note = MISC_FEATURE - Xaa is F3COO
  MOD_RES 14: note = METHYLATION
AVXVXNYXIIQXXYC

SEQ ID NO: 141 - protein, 15 aa, synthetic construct
  REGION 1..15: note = Synthesized polypeptide
  SITE 3: note = MISC_FEATURE - Xaa is MeF3C
  SITE 7: note = MISC_FEATURE - Xaa is 3Py6NH2
  SITE 8: note = MISC_FEATURE - Xaa is F4aao
  BINDING 11: note = PEG8Me
  SITE 13: note = MISC_FEATURE - Xaa is 4Py
  MOD_RES 14: note = METHYLATION
AVXVWNXXIIERXYC

SEQ ID NO: 142 - protein, 15 aa, synthetic construct
  REGION 1..15: note = Synthesized polypeptide
  MOD_RES 3: note = METHYLATION
  SITE 5: note = MISC_FEATURE - Xaa is W5C
  MOD_RES 14: note = METHYLATION
AVFVXNYYIIRRFFC

SEQ ID NO: 143 - protein, 15 aa, synthetic construct
  REGION 1..15: note = Synthesized polypeptide
  MOD_RES 3: note = METHYLATION
  SITE 5: note = MISC_FEATURE - Xaa is W5C
  SITE 8: note = MISC_FEATURE - Xaa is F4OMe
  MOD_RES 14: note = METHYLATION
AVFVXNYXIIRRFFC

SEQ ID NO: 144 - protein, 15 aa, synthetic construct
  REGION 1..15: note = Synthesized polypeptide
  MOD_RES 3: note = METHYLATION
  SITE 5: note = MISC_FEATURE - Xaa is W5C
  SITE 8: note = MISC_FEATURE - Xaa is F4OMe
  SITE 12: note = MISC_FEATURE - Xaa is dr
  MOD_RES 14: note = METHYLATION
AVFVXNYXIIRXFYC

SEQ ID NO: 145 - protein, 15 aa, synthetic construct
  REGION 1..15: note = Synthesized polypeptide
  SITE 3: note = MISC_FEATURE - Xaa is MeF4F
  SITE 5: note = MISC_FEATURE - Xaa is W5C
  SITE 8: note = MISC_FEATURE - Xaa is F4OMe
  MOD_RES 14: note = METHYLATION
AVXVXNYXIIRRFYC

SEQ ID NO: 146 - protein, 15 aa, synthetic construct
  REGION 1..15: note = Synthesized polypeptide
  SITE 3: note = MISC_FEATURE - Xaa is MeF4F
  SITE 5: note = MISC_FEATURE - Xaa is W5C
  SITE 8: note = MISC_FEATURE - Xaa is F4OMe
  SITE 12: note = MISC_FEATURE - Xaa is dr
  MOD_RES 14: note = METHYLATION
AVXVXNYXIIRXFYC

SEQ ID NO: 147 - protein, 15 aa, synthetic construct
  REGION 1..15: note = Synthesized polypeptide
  SITE 3: note = MISC_FEATURE - Xaa is Me4Py
  MOD_RES 5: note = METHYLATION
  SITE 8: note = MISC_FEATURE - Xaa is F4OMe
  SITE 12: note = MISC_FEATURE - Xaa is dr
  MOD_RES 14: note = METHYLATION
AVXVWNYXIIRXFYC

SEQ ID NO: 148 - protein, 15 aa, synthetic construct
  REGION 1..15: note = Synthesized polypeptide
  SITE 3: note = MISC_FEATURE - Xaa is MeF3COO
  MOD_RES 5: note = METHYLATION
  SITE 8: note = MISC_FEATURE - Xaa is F4OMe
  SITE 12: note = MISC_FEATURE - Xaa is dr
  MOD_RES 14: note = METHYLATION
AVXVWNYXIIRXFYC

SEQ ID NO: 149 - protein, 15 aa, synthetic construct
  REGION 1..15: note = Synthesized polypeptide
  MOD_RES 3: note = METHYLATION
  MOD_RES 14: note = METHYLATION
AVFVWAYYIIRRYYC

SEQ ID NO: 150 - protein, 15 aa, synthetic construct
  REGION 1..15: note = Synthesized polypeptide
  MOD_RES 3: note = METHYLATION
  SITE 5: note = MISC_FEATURE - Xaa is W5C
  MOD_RES 14: note = METHYLATION
AVFVXNYYIIRRYYC

SEQ ID NO: 151 - protein, 15 aa, synthetic construct
  REGION 1..15: note = Synthesized polypeptide
  MOD_RES 3: note = METHYLATION
  SITE 5: note = MISC_FEATURE - Xaa is W5C
  SITE 8: note = MISC_FEATURE - Xaa is F4OMe
  MOD_RES 14: note = METHYLATION
AVFVXNYXIIRRYYC

SEQ ID NO: 152 - protein, 15 aa, synthetic construct
  REGION 1..15: note = Synthesized polypeptide
  SITE 3: note = MISC_FEATURE - Xaa is MeF4F
  SITE 5: note = MISC_FEATURE - Xaa is W5C
  SITE 8: note = MISC_FEATURE - Xaa is F4OMe
  MOD_RES 14: note = METHYLATION
AVXVXNYXIIRRYYC

SEQ ID NO: 153 - protein, 15 aa, synthetic construct
  REGION 1..15: note = Synthesized polypeptide
  SITE 3: note = MISC_FEATURE - Xaa is MeF3C
  SITE 8: note = MISC_FEATURE - Xaa is F4OMe
  MOD_RES 14: note = METHYLATION
AVXVWNYXIIRRYYC

SEQ ID NO: 154 - protein, 15 aa, synthetic construct
  REGION 1..15: note = Synthesized polypeptide
  SITE 3: note = MISC_FEATURE - Xaa is MeF3C
  SITE 8: note = MISC_FEATURE - Xaa is F4OMe
  MOD_RES 14: note = METHYLATION
AVXVWNYXIIKRYYC

SEQ ID NO: 155 - protein, 15 aa, synthetic construct
  REGION 1..15: note = Synthesized polypeptide
  SITE 3: note = MISC_FEATURE - Xaa is MeF3C
  MOD_RES 5: note = METHYLATION
  SITE 8: note = MISC_FEATURE - Xaa is F4OMe
  MOD_RES 14: note = METHYLATION
AVXVWNYXIIRRYYC

SEQ ID NO: 156 - protein, 15 aa, synthetic construct
  REGION 1..15: note = Synthesized polypeptide
  MOD_RES 3: note = METHYLATION
  SITE 5: note = MISC_FEATURE - Xaa is W5C
  MOD_RES 14: note = METHYLATION
AVFVXNYYIIRRYYC

SEQ ID NO: 157 - protein, 15 aa, synthetic construct
  REGION 1..15: note = Synthesized polypeptide
  SITE 3: note = MISC_FEATURE - Xaa is MeF3C
  SITE 5: note = MISC_FEATURE - Xaa is W1aa
  SITE 8: note = MISC_FEATURE - Xaa is F4aao
  MOD_RES 14: note = METHYLATION
AVXVXNYXIIRRFYC

SEQ ID NO: 158 - protein, 15 aa, synthetic construct
  REGION 1..15: note = Synthesized polypeptide
  SITE 3: note = MISC_FEATURE - Xaa is MeF3C
  SITE 5: note = MISC_FEATURE - Xaa is W1aa
  SITE 8: note = MISC_FEATURE - Xaa is F4aao
  BINDING 11: note = PEG8Me
  MOD_RES 14: note = METHYLATION
AVXVXNYXIIERFYC

SEQ ID NO: 159 - protein, 15 aa, synthetic construct
  REGION 1..15: note = Synthesized polypeptide
  SITE 3: note = MISC_FEATURE - Xaa is MeF3C
  SITE 5: note = MISC_FEATURE - Xaa is W1aa
  SITE 8: note = MISC_FEATURE - Xaa is F4aao
  BINDING 12: note = PEG8Me
  MOD_RES 14: note = METHYLATION
AVXVXNYXIIREFYC

SEQ ID NO: 160 - protein, 15 aa, synthetic construct
  REGION 1..15: note = Synthesized polypeptide
  SITE 3: note = MISC_FEATURE - Xaa is MeF3C
  SITE 5: note = MISC_FEATURE - Xaa is W1aa
  SITE 8: note = MISC_FEATURE - Xaa is F4aao
  BINDING 11: note = PEG8Me
  BINDING 12: note = PEG8Me
  MOD_RES 14: note = METHYLATION
AVXVXNYXIIEEFYC

SEQ ID NO: 161 - protein, 15 aa, synthetic construct
  REGION 1..15: note = Synthesized polypeptide
  SITE 3: note = MISC_FEATURE - Xaa is MeF3C
  SITE 5: note = MISC_FEATURE - Xaa is W1aa
  SITE 8: note = MISC_FEATURE - Xaa is F4aao
  BINDING 11: note = PEG8Me
  SITE 13: note = MISC_FEATURE - Xaa is F3COO
  MOD_RES 14: note = METHYLATION
AVXVXNYXIIERXYC

SEQ ID NO: 162 - protein, 15 aa, synthetic construct
  REGION 1..15: note = Synthesized polypeptide
  SITE 3: note = MISC_FEATURE - Xaa is MeF3C
  SITE 5: note = MISC_FEATURE - Xaa is W1aa
  SITE 8: note = MISC_FEATURE - Xaa is F4aao
  MOD_RES 14: note = METHYLATION
AVXVXNYXIIQRFYC

SEQ ID NO: 163 - protein, 15 aa, synthetic construct
  REGION 1..15: note = Synthesized polypeptide
  SITE 3: note = MISC_FEATURE - Xaa is MeF3C
  SITE 5: note = MISC_FEATURE - Xaa is W1aa
  SITE 8: note = MISC_FEATURE - Xaa is F4aao
  MOD_RES 14: note = METHYLATION
AVXVXNYXIIRQFYC

SEQ ID NO: 164 - protein, 15 aa, synthetic construct
  REGION 1..15: note = Synthesized polypeptide
  SITE 3: note = MISC_FEATURE - Xaa is MeF3C
  SITE 5: note = MISC_FEATURE - Xaa is W1aa
  SITE 8: note = MISC_FEATURE - Xaa is F4aao
  MOD_RES 14: note = METHYLATION
AVXVXNYXIIQQFYC

SEQ ID NO: 165 - protein, 15 aa, synthetic construct
  REGION 1..15: note = Synthesized polypeptide
  SITE 3: note = MISC_FEATURE - Xaa is MeF3C
  SITE 5: note = MISC_FEATURE - Xaa is W1aa
  SITE 8: note = MISC_FEATURE - Xaa is F4OMe
  BINDING 11: note = PEG8Me
  BINDING 12: note = PEG8Me
  MOD_RES 14: note = METHYLATION
AVXVXNYXIEEEFYC

SEQ ID NO: 166 - protein, 15 aa, synthetic construct
  REGION 1..15: note = Synthesized polypeptide
  SITE 3: note = MISC_FEATURE - Xaa is MeF3C
  SITE 5: note = MISC_FEATURE - Xaa is W1aa
  SITE 8: note = MISC_FEATURE - Xaa is F4aao
  BINDING 11: note = PEG8Me
  BINDING 12: note = PEG8Me
  MOD_RES 14: note = METHYLATION
AVXVXNYXIIEEFYC

SEQ ID NO: 167 - protein, 15 aa, synthetic construct
  REGION 1..15: note = Synthesized polypeptide
  SITE 3: note = MISC_FEATURE - Xaa is MeF3C
  SITE 5: note = MISC_FEATURE - Xaa is W1aa
  SITE 8: note = MISC_FEATURE - Xaa is F4aao
  BINDING 11: note = PEG8Me
  BINDING 12: note = PEG8Me
  MOD_RES 14: note = METHYLATION
AVXVXNYXIIEEFYC

SEQ ID NO: 168 - protein, 15 aa, synthetic construct
  REGION 1..15: note = Synthesized polypeptide
  SITE 3: note = MISC_FEATURE - Xaa is MeF3C
  SITE 5: note = MISC_FEATURE - Xaa is W1aa
  SITE 8: note = MISC_FEATURE - Xaa is F4aao
  BINDING 11: note = PEG8Me
  BINDING 12: note = PEG8Me
  SITE 13: note = MISC_FEATURE - Xaa is F3COO
  MOD_RES 14: note = METHYLATION
AVXVXNYXIIEEXYC

SEQ ID NO: 169 - protein, 15 aa, synthetic construct
  REGION 1..15: note = Synthesized polypeptide
  SITE 3: note = MISC_FEATURE - Xaa is Me3Py
  SITE 7: note = MISC_FEATURE - Xaa is 3Py6NH2
  SITE 8: note = MISC_FEATURE - Xaa is 3Py
  SITE 13: note = MISC_FEATURE - Xaa is 4Py
  MOD_RES 14: note = METHYLATION
AVXVWNXXIIRRXYC

SEQ ID NO: 170 - protein, 15 aa, synthetic construct
  REGION 1..15: note = Synthesized polypeptide
  SITE 3: note = MISC_FEATURE - Xaa is MeF4F
  SITE 5: note = MISC_FEATURE - Xaa is W5C
  SITE 8: note = MISC_FEATURE - Xaa is F4OMe
  MOD_RES 14: note = METHYLATION
AVXVXNYXIIRRYYC

SEQ ID NO: 171 - protein, 15 aa, synthetic construct
  REGION 1..15: note = Synthesized polypeptide
  SITE 3: note = MISC_FEATURE - Xaa is MeF3C
  SITE 8: note = MISC_FEATURE - Xaa is F4OMe
  MOD_RES 14: note = METHYLATION
AVXVWNYXIIKRYYC

SEQ ID NO: 172 - protein, 15 aa, synthetic construct
  REGION 1..15: note = Synthesized polypeptide
  SITE 3: note = MISC_FEATURE - Xaa is MeF3C
  MOD_RES 5: note = METHYLATION
  SITE 8: note = MISC_FEATURE - Xaa is F4OMe
  MOD_RES 14: note = METHYLATION
AVXVWNYXIIRRYYC

SEQ ID NO: 173 - protein, 15 aa, synthetic construct
  REGION 1..15: note = Synthesized polypeptide
  SITE 3: note = MISC_FEATURE - Xaa is MeF3C
  SITE 8: note = MISC_FEATURE - Xaa is 3Py
  BINDING 11: note = PEG1Me
  BINDING 12: note = PEG1Me
  SITE 13: note = MISC_FEATURE - Xaa is 4Py
  MOD_RES 14: note = METHYLATION
AVXVWNYXIIEEXYC

SEQ ID NO: 174 - protein, 15 aa, synthetic construct
  REGION 1..15: note = Synthesized polypeptide
  SITE 3: note = MISC_FEATURE - Xaa is MeF3C
  SITE 8: note = MISC_FEATURE - Xaa is 3Py
  BINDING 11: note = Glucamine
  BINDING 12: note = Glucamine
  SITE 13: note = MISC_FEATURE - Xaa is 4Py
  MOD_RES 14: note = METHYLATION
AVXVWNYXIIEEXYC

SEQ ID NO: 175 - protein, 15 aa, synthetic construct
  REGION 1..15: note = Synthesized polypeptide
  SITE 3: note = MISC_FEATURE - Xaa is MeF3C
  SITE 5: note = MISC_FEATURE - Xaa is W1aa
  SITE 8: note = MISC_FEATURE - Xaa is F4aao
  BINDING 11: note = PEG1Me
  BINDING 12: note = PEG1Me
  SITE 13: note = MISC_FEATURE - Xaa is F3COO
  MOD_RES 14: note = METHYLATION
AVXVXNYXIIEEXYC

SEQ ID NO: 176 - protein, 15 aa, synthetic construct
  REGION 1..15: note = Synthesized polypeptide
  SITE 3: note = MISC_FEATURE - Xaa is MeF3C
  SITE 8: note = MISC_FEATURE - Xaa is F4OMe
  BINDING 11: note = PEG1Me
  BINDING 12: note = PEG1Me
  MOD_RES 14: note = METHYLATION
AVXVWNYXIIEEFYC

SEQ ID NO: 177 - protein, 15 aa, synthetic construct
  REGION 1..15: note = Synthesized polypeptide
  SITE 3: note = MISC_FEATURE - Xaa is MeF3C
  SITE 8: note = MISC_FEATURE - Xaa is F4OMe
  MOD_RES 14: note = METHYLATION
AVXVWNYXIIQQFYC

SEQ ID NO: 178 - protein, 15 aa, synthetic construct
  REGION 1..15: note = Synthesized polypeptide
  SITE 3: note = MISC_FEATURE - Xaa is MeF3C
  SITE 5: note = MISC_FEATURE - Xaa is W1aa
  SITE 8: note = MISC_FEATURE - Xaa is 3Py
  SITE 13: note = MISC_FEATURE - Xaa is 4Py
  MOD_RES 14: note = METHYLATION
AVXVXNYXIIRRXYC

SEQ ID NO: 179 - protein, 15 aa, synthetic construct
  REGION 1..15: note = Synthesized polypeptide
  SITE 3: note = MISC_FEATURE - Xaa is MeF3C
  SITE 5: note = MISC_FEATURE - Xaa is W1aa
  SITE 7: note = MISC_FEATURE - Xaa is 3Py6NH2
  SITE 8: note = MISC_FEATURE - Xaa is 3Py
  SITE 13: note = MISC_FEATURE - Xaa is 4Py
  MOD_RES 14: note = METHYLATION
AVXVXNXXIIRRXYC

SEQ ID NO: 180 - protein, 15 aa, synthetic construct
  REGION 1..15: note = Synthesized polypeptide
  SITE 3: note = MISC_FEATURE - Xaa is MeF3C
  SITE 5: note = MISC_FEATURE - Xaa is W1aa
  SITE 7: note = MISC_FEATURE - Xaa is 3Py6NH2
  SITE 8: note = MISC_FEATURE - Xaa is F4OMe
  SITE 13: note = MISC_FEATURE - Xaa is 4Py
  MOD_RES 14: note = METHYLATION
AVXVXNXXIIRRXYC

SEQ ID NO: 181 - protein, 15 aa, synthetic construct
  REGION 1..15: note = Synthesized polypeptide
  SITE 3: note = MISC_FEATURE - Xaa is MeF3C
  SITE 8: note = MISC_FEATURE - Xaa is 3Py
  SITE 13: note = MISC_FEATURE - Xaa is 4Py
  MOD_RES 14: note = METHYLATION
AVXVWNYXIIRRXYC

SEQ ID NO: 182 - protein, 15 aa, synthetic construct
  REGION 1..15: note = Synthesized polypeptide
  SITE 3: note = MISC_FEATURE - Xaa is MeF3C
  SITE 7: note = MISC_FEATURE - Xaa is 3Py6NH2
  SITE 8: note = MISC_FEATURE - Xaa is 3Py
  SITE 13: note = MISC_FEATURE - Xaa is 4Py
  MOD_RES 14: note = METHYLATION
AVXVWNXXIIRRXYC

SEQ ID NO: 183 - protein, 15 aa, synthetic construct
  REGION 1..15: note = Synthesized polypeptide
  SITE 3: note = MISC_FEATURE - Xaa is MeF3C
  SITE 7: note = MISC_FEATURE - Xaa is 3Py6NH2
  SITE 8: note = MISC_FEATURE - Xaa is F4OMe
  SITE 13: note = MISC_FEATURE - Xaa is 4Py
  MOD_RES 14: note = METHYLATION
AVXVWNXXIIRRXYC

SEQ ID NO: 184 - protein, 15 aa, synthetic construct
  REGION 1..15: note = Synthesized polypeptide
  SITE 3: note = MISC_FEATURE - Xaa is MeF3C
  SITE 8: note = MISC_FEATURE - Xaa is 4Py
  SITE 13: note = MISC_FEATURE - Xaa is 4Py
  MOD_RES 14: note = METHYLATION
AVXVWNYXIIRRXYC

SEQ ID NO: 185 - protein, 15 aa, synthetic construct
  REGION 1..15: note = Synthesized polypeptide
  SITE 3: note = MISC_FEATURE - Xaa is MeF3C
  SITE 5: note = MISC_FEATURE - Xaa is W1aa
  SITE 7: note = MISC_FEATURE - Xaa is 3Py6NH2
  SITE 8: note = MISC_FEATURE - Xaa is F4OMe
  MOD_RES 14: note = METHYLATION
AVXVXNXXIIRRFYC

SEQ ID NO: 186 - protein, 15 aa, synthetic construct
  REGION 1..15: note = Synthesized polypeptide
  SITE 3: note = MISC_FEATURE - Xaa is MeF3C
  SITE 5: note = MISC_FEATURE - Xaa is W1aa
  SITE 8: note = MISC_FEATURE - Xaa is 3Py
  MOD_RES 14: note = METHYLATION
AVXVXNYXIIRRFYC

SEQ ID NO: 187 - protein, 15 aa, synthetic construct
  REGION 1..15: note = Synthesized polypeptide
  SITE 3: note = MISC_FEATURE - Xaa is MeF3C
  SITE 5: note = MISC_FEATURE - Xaa is W1aa
  SITE 8: note = MISC_FEATURE - Xaa is F4OMe
  SITE 13: note = MISC_FEATURE - Xaa is 4Py
  MOD_RES 14: note = METHYLATION
AVXVXNYXIIRRXYC

SEQ ID NO: 188 - protein, 15 aa, synthetic construct
  REGION 1..15: note = Synthesized polypeptide
  SITE 3: note = MISC_FEATURE - Xaa is MeF3C
  SITE 5: note = MISC_FEATURE - Xaa is W1aa
  SITE 8: note = MISC_FEATURE - Xaa is F4OMe
  SITE 13: note = MISC_FEATURE - Xaa is F3COO
  MOD_RES 14: note = METHYLATION
AVXVXNYXIIRRXYC

SEQ ID NO: 189 - protein, 15 aa, synthetic construct
  REGION 1..15: note = Synthesized polypeptide
  SITE 3: note = MISC_FEATURE - Xaa is MeF3C
  SITE 5: note = MISC_FEATURE - Xaa is W1aa
  SITE 7: note = MISC_FEATURE - Xaa is 3Py6NH2
  SITE 8: note = MISC_FEATURE - Xaa is 3Py
  MOD_RES 14: note = METHYLATION
AVXVXNXXIIRRFYC

SEQ ID NO: 190 - protein, 15 aa, synthetic construct
  REGION 1..15: note = Synthesized polypeptide
  SITE 3: note = MISC_FEATURE - Xaa is MeF3C
  SITE 7: note = MISC_FEATURE - Xaa is 3Py6NH2
  SITE 8: note = MISC_FEATURE - Xaa is 3Py
  MOD_RES 14: note = METHYLATION
AVXVWNXXIIRRFYC

SEQ ID NO: 191 - protein, 15 aa, synthetic construct
  REGION 1..15: note = Synthesized polypeptide
  SITE 3: note = MISC_FEATURE - Xaa is MeF3C
  SITE 7: note = MISC_FEATURE - Xaa is 3Py6NH2
  SITE 8: note = MISC_FEATURE - Xaa is F4aao
  MOD_RES 14: note = METHYLATION
AVXVWNXXIIRRFYC

SEQ ID NO: 192 - protein, 15 aa, synthetic construct
  REGION 1..15: note = Synthesized polypeptide
  SITE 3: note = MISC_FEATURE - Xaa is MeF3C
  SITE 7: note = MISC_FEATURE - Xaa is 3Py6NH2
  SITE 8: note = MISC_FEATURE - Xaa is F4OMe
  SITE 13: note = MISC_FEATURE - Xaa is F3COO
  MOD_RES 14: note = METHYLATION
AVXVWNXXIIRRXYC

SEQ ID NO: 193 - protein, 15 aa, synthetic construct
  REGION 1..15: note = Synthesized polypeptide
  SITE 3: note = MISC_FEATURE - Xaa is MeF3C
  SITE 8: note = MISC_FEATURE - Xaa is 3Py
  BINDING 12: note = PEG8Me
  MOD_RES 14: note = METHYLATION
AVXVWNYXIIREFYC

SEQ ID NO: 194 - protein, 15 aa, synthetic construct
  REGION 1..15: note = Synthesized polypeptide
  SITE 3: note = MISC_FEATURE - Xaa is MeF3C
  SITE 8: note = MISC_FEATURE - Xaa is 3Py
  SITE 13: note = MISC_FEATURE - Xaa is F3COO
  MOD_RES 14: note = METHYLATION
AVXVWNYXIIRRXYC

SEQ ID NO: 195 - protein, 15 aa, synthetic construct
  REGION 1..15: note = Synthesized polypeptide
  SITE 3: note = MISC_FEATURE - Xaa is MeF3C
  SITE 8: note = MISC_FEATURE - Xaa is F4aao
  SITE 13: note = MISC_FEATURE - Xaa is F3COO
  MOD_RES 14: note = METHYLATION
AVXVWNYXIIRRXYC

SEQ ID NO: 196 - protein, 15 aa, synthetic construct
  REGION 1..15: note = Synthesized polypeptide
  SITE 3: note = MISC_FEATURE - Xaa is MeF3C
  SITE 8: note = MISC_FEATURE - Xaa is F4aao
  SITE 13: note = MISC_FEATURE - Xaa is 4Py
  MOD_RES 14: note = METHYLATION
AVXVWNYXIIRRXYC

SEQ ID NO: 197 - protein, 15 aa, synthetic construct
  REGION 1..15: note = Synthesized polypeptide
  SITE 3: note = MISC_FEATURE - Xaa is MeF3C
  SITE 8: note = MISC_FEATURE - Xaa is F4OMe
  BINDING 12: note = PEG8Me
  SITE 13: note = MISC_FEATURE - Xaa is 4Py
  MOD_RES 14: note = METHYLATION
AVXVWNYXIIREXYC

SEQ ID NO: 198 - protein, 15 aa, synthetic construct
  REGION 1..15: note = Synthesized polypeptide
  SITE 3: note = MISC_FEATURE - Xaa is MeF3C
  SITE 7: note = MISC_FEATURE - Xaa is 3Py6NH2
  SITE 8: note = MISC_FEATURE - Xaa is 3Py
  SITE 13: note = MISC_FEATURE - Xaa is F3COO
  MOD_RES 14: note = METHYLATION
AVXVWNXXIIRRXYC

SEQ ID NO: 199 - protein, 15 aa, synthetic construct
  REGION 1..15: note = Synthesized polypeptide
  SITE 3: note = MISC_FEATURE - Xaa is MeF3C
  SITE 5: note = MISC_FEATURE - Xaa is W1aa
  SITE 8: note = MISC_FEATURE - Xaa is F4aao
  BINDING 11: note = Mecar
  MOD_RES 14: note = METHYLATION
AVXVXNYXIIKRFYC

SEQ ID NO: 200 - protein, 15 aa, synthetic construct
  REGION 1..15: note = Synthesized polypeptide
  SITE 3: note = MISC_FEATURE - Xaa is MeF3C
  SITE 5: note = MISC_FEATURE - Xaa is W1aa
  SITE 8: note = MISC_FEATURE - Xaa is F4aao
  BINDING 12: note = Mecar
  MOD_RES 14: note = METHYLATION
AVXVXNYXIIRKFYC

SEQ ID NO: 201 - protein, 15 aa, synthetic construct
  REGION 1..15: note = Synthesized polypeptide
  SITE 3: note = MISC_FEATURE - Xaa is MeF3C
  SITE 5: note = MISC_FEATURE - Xaa is W1aa
  SITE 8: note = MISC_FEATURE - Xaa is F4aao
  SITE 11: note = MISC_FEATURE - Xaa is QhEt
  MOD_RES 14: note = METHYLATION
AVXVXNYXIIXRFYC

SEQ ID NO: 202 - protein, 15 aa, synthetic construct
  REGION 1..15: note = Synthesized polypeptide
  SITE 3: note = MISC_FEATURE - Xaa is MeF3C
  SITE 5: note = MISC_FEATURE - Xaa is W1aa
  SITE 8: note = MISC_FEATURE - Xaa is F4aao
  SITE 12: note = MISC_FEATURE - Xaa is QhEt
  MOD_RES 14: note = METHYLATION
AVXVXNYXIIRXFYC

SEQ ID NO: 203 - protein, 15 aa, synthetic construct
  REGION 1..15: note = Synthesized polypeptide
  SITE 3: note = MISC_FEATURE - Xaa is MeF3C
  SITE 5: note = MISC_FEATURE - Xaa is W1aa
  SITE 8: note = MISC_FEATURE - Xaa is F4aao
  SITE 11: note = MISC_FEATURE - Xaa is QhEt
  SITE 12: note = MISC_FEATURE - Xaa is QhEt
  MOD_RES 14: note = METHYLATION
AVXVXNYXIIXXFYC

SEQ ID NO: 204 - protein, 15 aa, synthetic construct
  REGION 1..15: note = Synthesized polypeptide
  SITE 3: note = MISC_FEATURE - Xaa is MeF3C
  SITE 5: note = MISC_FEATURE - Xaa is W1aa
  SITE 8: note = MISC_FEATURE - Xaa is F4aao
  SITE 11: note = MISC_FEATURE - Xaa is Qpipzaa
  MOD_RES 14: note = METHYLATION
AVXVXNYXIIXRFYC

SEQ ID NO: 205 - protein, 15 aa, synthetic construct
  REGION 1..15: note = Synthesized polypeptide
  SITE 3: note = MISC_FEATURE - Xaa is MeF3C
  SITE 5: note = MISC_FEATURE - Xaa is W1aa
  SITE 8: note = MISC_FEATURE - Xaa is F4aao
  SITE 12: note = MISC_FEATURE - Xaa is Qpipzaa
  MOD_RES 14: note = METHYLATION
AVXVXNYXIIRXFYC

SEQ ID NO: 206 - protein, 15 aa, synthetic construct
  REGION 1..15: note = Synthesized polypeptide
  SITE 3: note = MISC_FEATURE - Xaa is MeF3C
  SITE 5: note = MISC_FEATURE - Xaa is W1aa
  SITE 8: note = MISC_FEATURE - Xaa is F4aao
  SITE 11: note = MISC_FEATURE - Xaa is Qpipzaa
  SITE 12: note = MISC_FEATURE - Xaa is Qpipzaa
  MOD_RES 14: note = METHYLATION
AVXVXNYXIIXXFYC

SEQ ID NO: 207 - protein, 15 aa, synthetic construct
  REGION 1..15: note = Synthesized polypeptide
  SITE 3: note = MISC_FEATURE - Xaa is MeF3C
  SITE 5: note = MISC_FEATURE - Xaa is W1aa
  SITE 8: note = MISC_FEATURE - Xaa is F4aao
  SITE 11: note = MISC_FEATURE - Xaa is A4paa
  MOD_RES 14: note = METHYLATION
AVXVXNYXIIXRFYC

SEQ ID NO: 208 - protein, 15 aa, synthetic construct
  REGION 1..15: note = Synthesized polypeptide
  SITE 3: note = MISC_FEATURE - Xaa is MeF3C
  SITE 5: note = MISC_FEATURE - Xaa is W1aa
  SITE 8: note = MISC_FEATURE - Xaa is F4aao
  SITE 12: note = MISC_FEATURE - Xaa is A4paa
  MOD_RES 14: note = METHYLATION
AVXVXNYXIIRXFYC

SEQ ID NO: 209 - protein, 15 aa, synthetic construct
  REGION 1..15: note = Synthesized polypeptide
  SITE 3: note = MISC_FEATURE - Xaa is MeF3C
  SITE 5: note = MISC_FEATURE - Xaa is W1aa
  SITE 8: note = MISC_FEATURE - Xaa is F4aao
  SITE 11: note = MISC_FEATURE - Xaa is Kmor
  MOD_RES 14: note = METHYLATION
AVXVXNYXIIXRFYC

SEQ ID NO: 210 - protein, 15 aa, synthetic construct
  REGION 1..15: note = Synthesized polypeptide
  SITE 3: note = MISC_FEATURE - Xaa is MeF3C
  SITE 5: note = MISC_FEATURE - Xaa is W1aa
  SITE 8: note = MISC_FEATURE - Xaa is F4aao
  SITE 12: note = MISC_FEATURE - Xaa is Kmor
  MOD_RES 14: note = METHYLATION
AVXVXNYXIIRXFYC

SEQ ID NO: 211 - protein, 15 aa, synthetic construct
  REGION 1..15: note = Synthesized polypeptide
  SITE 3: note = MISC_FEATURE - Xaa is MeF3C
  SITE 5: note = MISC_FEATURE - Xaa is W1aa
  SITE 8: note = MISC_FEATURE - Xaa is F4aao
  SITE 11: note = MISC_FEATURE - Xaa is Kmor
  SITE 12: note = MISC_FEATURE - Xaa is Kmor
  MOD_RES 14: note = METHYLATION
AVXVXNYXIIXXFYC

SEQ ID NO: 212 - protein, 15 aa, synthetic construct
  REGION 1..15: note = Synthesized polypeptide
  SITE 3: note = MISC_FEATURE - Xaa is MeF3C
  SITE 5: note = MISC_FEATURE - Xaa is W1aa
  SITE 8: note = MISC_FEATURE - Xaa is F4aao
  MOD_RES 14: note = METHYLATION
AVXVXNYXIIRRFYC

SEQ ID NO: 213 - protein, 15 aa, synthetic construct
  REGION 1..15: note = Synthesized polypeptide
  SITE 3: note = MISC_FEATURE - Xaa is MeF3C
  SITE 5: note = MISC_FEATURE - Xaa is W1aa
  SITE 8: note = MISC_FEATURE - Xaa is F4aao
  MOD_RES 14: note = METHYLATION
AVXVXNYXIIRRFYC

SEQ ID NO: 214 - protein, 15 aa, synthetic construct
  REGION 1..15: note = Synthesized polypeptide
  SITE 3: note = MISC_FEATURE - Xaa is MeF3C
  SITE 5: note = MISC_FEATURE - Xaa is W1aa
  SITE 8: note = MISC_FEATURE - Xaa is F4aao
  BINDING 11: note = PEG8Me
  MOD_RES 14: note = METHYLATION
AVXVXNYXIIERFYC

SEQ ID NO: 215 - protein, 15 aa, synthetic construct
  REGION 1..15: note = Synthesized polypeptide
  MOD_RES 3: note = METHYLATION
  MOD_RES 5: note = METHYLATION
  MOD_RES 14: note = METHYLATION
AVFVWNYYIIKRYYC

SEQ ID NO: 216 - protein, 15 aa, synthetic construct
  REGION 1..15: note = Synthesized polypeptide
  SITE 3: note = MISC_FEATURE - Xaa is MeF3C
  SITE 5: note = MISC_FEATURE - Xaa is W1aa
  SITE 8: note = MISC_FEATURE - Xaa is F4aao
  SITE 12: note = MISC_FEATURE - Xaa is Kmor
  SITE 13: note = MISC_FEATURE - Xaa is F3COO
  MOD_RES 14: note = METHYLATION
AVXVXNYXIIQXXYC

SEQ ID NO: 217 - protein, 15 aa, synthetic construct
  REGION 1..15: note = Synthesized polypeptide
  SITE 3: note = MISC_FEATURE - Xaa is MeF3C
  SITE 5: note = MISC_FEATURE - Xaa is W1aa
  SITE 8: note = MISC_FEATURE - Xaa is F4aao
  BINDING 11: note = PEG8Me
  SITE 12: note = MISC_FEATURE - Xaa is Kmor
  SITE 13: note = MISC_FEATURE - Xaa is F3COO
  MOD_RES 14: note = METHYLATION
AVXVXNYXIIEXXYC

SEQ ID NO: 218 - protein, 15 aa, synthetic construct
  REGION 1..15: note = Synthesized polypeptide
  SITE 3: note = MISC_FEATURE - Xaa is MeF3C
  SITE 5: note = MISC_FEATURE - Xaa is W7N
  SITE 8: note = MISC_FEATURE - Xaa is F4aao
  BINDING 11: note = PEG8Me
  SITE 13: note = MISC_FEATURE - Xaa is 4Py
  MOD_RES 14: note = METHYLATION
AVXVXNYXIIERXYC

SEQ ID NO: 219 - protein, 15 aa, synthetic construct
  REGION 1..15: note = Synthesized polypeptide
  SITE 3: note = MISC_FEATURE - Xaa is MeF3C
  SITE 5: note = MISC_FEATURE - Xaa is W1aa
  SITE 8: note = MISC_FEATURE - Xaa is F4aao
  BINDING 11: note = PEG8Me
  SITE 12: note = MISC_FEATURE - Xaa is Kmor
  SITE 13: note = MISC_FEATURE - Xaa is 4Py
  MOD_RES 14: note = METHYLATION
AVXVXNYXIIEXXYC

SEQ ID NO: 220 - protein, 15 aa, synthetic construct
  REGION 1..15: note = Synthesized polypeptide
  SITE 3: note = MISC_FEATURE - Xaa is MeF3C
  SITE 5: note = MISC_FEATURE - Xaa is W7N
  SITE 8: note = MISC_FEATURE - Xaa is F4aao
  BINDING 11: note = PEG8Me
  SITE 12: note = MISC_FEATURE - Xaa is Kmor
  SITE 13: note = MISC_FEATURE - Xaa is F3COO
  MOD_RES 14: note = METHYLATION
AVXVXNYXIIEXXYC

SEQ ID NO: 221 - protein, 15 aa, synthetic construct
  REGION 1..15: note = Synthesized polypeptide
  SITE 3: note = MISC_FEATURE - Xaa is MeF3C
  SITE 5: note = MISC_FEATURE - Xaa is W7N
  SITE 8: note = MISC_FEATURE - Xaa is F4aao
  BINDING 11: note = PEG8Me
  BINDING 13: note = PEG8Me
  MOD_RES 14: note = METHYLATION
AVXVXNYXIIEREYC

SEQ ID NO: 222 - protein, 15 aa, synthetic construct
  REGION 1..15: note = Synthesized polypeptide
  SITE 3: note = MISC_FEATURE - Xaa is MeF3C
  SITE 5: note = MISC_FEATURE - Xaa is W1aa
  SITE 7: note = MISC_FEATURE - Xaa is 3Py6NH2
  SITE 8: note = MISC_FEATURE - Xaa is F4aao
  BINDING 11: note = PEG8Me
  SITE 13: note = MISC_FEATURE - Xaa is 4Py
  MOD_RES 14: note = METHYLATION
AVXVXNXXIIERXYC

SEQ ID NO: 223 - protein, 15 aa, synthetic construct
  REGION 1..15: note = Synthesized polypeptide
  SITE 3: note = MISC_FEATURE - Xaa is MeF3C
  SITE 5: note = MISC_FEATURE - Xaa is W1aa
  SITE 7: note = MISC_FEATURE - Xaa is 3Py6NH2
  SITE 8: note = MISC_FEATURE - Xaa is F4aao
  BINDING 11: note = PEG8Me
  SITE 13: note = MISC_FEATURE - Xaa is F3COO
  MOD_RES 14: note = METHYLATION
AVXVXNXXIIERXYC

SEQ ID NO: 224 - protein, 15 aa, synthetic construct
  REGION 1..15: note = Synthesized polypeptide
  SITE 3: note = MISC_FEATURE - Xaa is MeF3C
  SITE 5: note = MISC_FEATURE - Xaa is W7N
  SITE 7: note = MISC_FEATURE - Xaa is 3Py6NH2
  SITE 8: note = MISC_FEATURE - Xaa is F4aao
  BINDING 11: note = PEG8Me
  SITE 13: note = MISC_FEATURE - Xaa is 4Py
  MOD_RES 14: note = METHYLATION
AVXVXNXXIIERXYC

SEQ ID NO: 225 - protein, 15 aa, synthetic construct
  REGION 1..15: note = Synthesized polypeptide
  SITE 3: note = MISC_FEATURE - Xaa is MeF3C
  SITE 5: note = MISC_FEATURE - Xaa is W7N
  SITE 8: note = MISC_FEATURE - Xaa is F4aao
  SITE 13: note = MISC_FEATURE - Xaa is F3COO
  MOD_RES 14: note = METHYLATION
AVXVXNYXIIQRXYC

SEQ ID NO: 226 - protein, 15 aa, synthetic construct
  REGION 1..15: note = Synthesized polypeptide
  SITE 3: note = MISC_FEATURE - Xaa is MeF3C
  SITE 5: note = MISC_FEATURE - Xaa is W7N
  SITE 8: note = MISC_FEATURE - Xaa is F4aao(PEG8Me)
  SITE 13: note = MISC_FEATURE - Xaa is F3COO(PEG8Me)
  SITE 14: note = MISC_FEATURE - Xaa is MeF4COO(PEG8Me)
AVXVXNYXIIQQXXC

SEQ ID NO: 227 - protein, 15 aa, synthetic construct
  REGION 1..15: note = Synthesized polypeptide
  SITE 3: note = MISC_FEATURE - Xaa is MeF3C
  SITE 5: note = MISC_FEATURE - Xaa is W7N
  SITE 8: note = MISC_FEATURE - Xaa is F4aao(PEG8Me)
  SITE 13: note = MISC_FEATURE - Xaa is 4Py
  SITE 14: note = MISC_FEATURE - Xaa is MeF4COO(PEG8Me)
AVXVXNYXIIQQXXC

SEQ ID NO: 228 - protein, 15 aa, synthetic construct
  REGION 1..15: note = Synthesized polypeptide
  SITE 3: note = MISC_FEATURE - Xaa is MeF3C
  SITE 5: note = MISC_FEATURE - Xaa is W7N
  SITE 8: note = MISC_FEATURE - Xaa is F4OMe
  SITE 13: note = MISC_FEATURE - Xaa is F3COO(PEG8Me)
  SITE 14: note = MISC_FEATURE - Xaa is MeF4COO(PEG8Me)
AVXVXNYXIIQQXXC

SEQ ID NO: 229 - protein, 15 aa, synthetic construct
  REGION 1..15: note = Synthesized polypeptide
  SITE 3: note = MISC_FEATURE - Xaa is MeF3C
  SITE 5: note = MISC_FEATURE - Xaa is W7N
  SITE 8: note = MISC_FEATURE - Xaa is F4aao(PEG8Me)
  SITE 13: note = MISC_FEATURE - Xaa is F3COO(PEG8Me)
  MOD_RES 14: note = METHYLATION
AVXVXNYXIIQQXYC

SEQ ID NO: 230 - protein, 15 aa, synthetic construct
  REGION 1..15: note = Synthesized polypeptide
  SITE 3: note = MISC_FEATURE - Xaa is MeF3C
  SITE 5: note = MISC_FEATURE - Xaa is W7N
  SITE 8: note = MISC_FEATURE - Xaa is F4aao
  BINDING 11: note = PEG8Me
  SITE 13: note = MISC_FEATURE - Xaa is F3COO
  MOD_RES 14: note = METHYLATION
AVXVXNYXIIERXYC

SEQ ID NO: 231 - protein, 15 aa, synthetic construct
  REGION 1..15: note = Synthesized polypeptide
  SITE 3: note = MISC_FEATURE - Xaa is MeF3C
  SITE 5: note = MISC_FEATURE - Xaa is W1aa
  SITE 8: note = MISC_FEATURE - Xaa is F4aao
  BINDING 11: note = PEG8Me
  SITE 13: note = MISC_FEATURE - Xaa is 4Py
  MOD_RES 14: note = METHYLATION
AVXVXNYXIIERXYC

SEQ ID NO: 232 - protein, 15 aa, synthetic construct
  REGION 1..15: note = Synthesized polypeptide
  SITE 3: note = MISC_FEATURE - Xaa is MeF3C
  SITE 5: note = MISC_FEATURE - Xaa is W7N
  SITE 7: note = MISC_FEATURE - Xaa is 3Py6NH2
  SITE 8: note = MISC_FEATURE - Xaa is F4aao
  BINDING 11: note = PEG8Me
  BINDING 13: note = PEG8Me
  MOD_RES 14: note = METHYLATION
AVXVXNXXIIEREYC

SEQ ID NO: 233 - protein, 15 aa, synthetic construct
  REGION 1..15: note = Synthesized polypeptide
  SITE 3: note = MISC_FEATURE - Xaa is MeF3C
  SITE 5: note = MISC_FEATURE - Xaa is W7N
  SITE 7: note = MISC_FEATURE - Xaa is 3Py6NH2
  SITE 8: note = MISC_FEATURE - Xaa is F4aao
  BINDING 11: note = PEG8Me
  SITE 12: note = MISC_FEATURE - Xaa is Kmor
  SITE 13: note = MISC_FEATURE - Xaa is F3COO
  MOD_RES 14: note = METHYLATION
AVXVXNXXIIEXXYC

SEQ ID NO: 234 - protein, 15 aa, synthetic construct
  REGION 1..15: note = Synthesized polypeptide
  SITE 3: note = MISC_FEATURE - Xaa is MeF3C
  SITE 5: note = MISC_FEATURE - Xaa is W7N
  SITE 8: note = MISC_FEATURE - Xaa is F4aao
  BINDING 11: note = PEG8Me
  SITE 12: note = MISC_FEATURE - Xaa is Kmor
  BINDING 13: note = PEG8Me
  MOD_RES 14: note = METHYLATION
AVXVXNYXIIEXEYC

SEQ ID NO: 235 - protein, 15 aa, synthetic construct
  REGION 1..15: note = Synthesized polypeptide
  SITE 3: note = MISC_FEATURE - Xaa is MeF3C
  SITE 5: note = MISC_FEATURE - Xaa is W7N
  SITE 8: note = MISC_FEATURE - Xaa is F4OMe
  BINDING 11: note = PEG8Me
  SITE 12: note = MISC_FEATURE - Xaa is Kmor
  BINDING 13: note = PEG8Me
  MOD_RES 14: note = METHYLATION
AVXVXNYXIIEXEYC

SEQ ID NO: 236 - protein, 15 aa, synthetic construct
  REGION 1..15: note = Synthesized polypeptide
  SITE 3: note = MISC_FEATURE - Xaa is MeF3C
  SITE 5: note = MISC_FEATURE - Xaa is W7N
  SITE 7: note = MISC_FEATURE - Xaa is 3Py6NH2
  SITE 8: note = MISC_FEATURE - Xaa is F4OMe
  BINDING 11: note = PEG8Me
  SITE 12: note = MISC_FEATURE - Xaa is Kmor
  SITE 13: note = MISC_FEATURE - Xaa is 4Py
  MOD_RES 14: note = METHYLATION
AVXVXNXXIIEXXYC

SEQ ID NO: 237 - protein, 15 aa, synthetic construct
  REGION 1..15: note = Synthesized polypeptide
  SITE 3: note = MISC_FEATURE - Xaa is MeF3C
  SITE 5: note = MISC_FEATURE - Xaa is W7N
  SITE 7: note = MISC_FEATURE - Xaa is 3Py6NH2
  SITE 8: note = MISC_FEATURE - Xaa is F4OMe
  BINDING 11: note = PEG8Me
  SITE 12: note = MISC_FEATURE - Xaa is KCOpipzaa
  SITE 13: note = MISC_FEATURE - Xaa is 4Py
  MOD_RES 14: note = METHYLATION
AVXVXNXXIIEXXYC

SEQ ID NO: 238 - protein, 15 aa, synthetic construct
  REGION 1..15: note = Synthesized polypeptide
  SITE 3: note = MISC_FEATURE - Xaa is MeF3C
  SITE 7: note = MISC_FEATURE - Xaa is 3Py6NH2
  SITE 8: note = MISC_FEATURE - Xaa is F4aao
  BINDING 11: note = PEG8Me
  SITE 13: note = MISC_FEATURE - Xaa is F3COO
  MOD_RES 14: note = METHYLATION
AVXVWNXXIIERXYC

SEQ ID NO: 239 - protein, 15 aa, synthetic construct
  REGION 1..15: note = Synthesized polypeptide
  SITE 3: note = MISC_FEATURE - Xaa is MeF3C
  SITE 5: note = MISC_FEATURE - Xaa is W7N
  SITE 7: note = MISC_FEATURE - Xaa is 3Py6NH2
  SITE 8: note = MISC_FEATURE - Xaa is F4aao
  BINDING 11: note = PEG8Me
  SITE 13: note = MISC_FEATURE - Xaa is F3COO
  MOD_RES 14: note = METHYLATION
AVXVXNXXIIERXYC

SEQ ID NO: 240 - protein, 15 aa, synthetic construct
  REGION 1..15: note = Synthesized polypeptide
  SITE 3: note = MISC_FEATURE - Xaa is MeF3C
  SITE 5: note = MISC_FEATURE - Xaa is W1aa
  SITE 8: note = MISC_FEATURE - Xaa is F4aao
  SITE 11: note = MISC_FEATURE - Xaa is Kmor
  SITE 12: note = MISC_FEATURE - Xaa is Kmor
  SITE 13: note = MISC_FEATURE - Xaa is F3COO
  MOD_RES 14: note = METHYLATION
AVXVXNYXIIXXXYC

SEQ ID NO: 241 - protein, 15 aa, synthetic construct
  REGION 1..15: note = Synthesized polypeptide
  MOD_RES 3: note = METHYLATION
  MOD_RES 5: note = METHYLATION
  MOD_RES 14: note = METHYLATION
AVFVWNYYIIKRYYC

SEQ ID NO: 242-245 - skipped (4 entries)

SEQ ID NO: 246 - protein, 7 aa, synthetic construct
  REGION 1..7: note = Synthesized polypeptide
  SITE 2: note = MISC_FEATURE - Xaa is de
  SITE 3: note = MISC_FEATURE - Xaa is de
  SITE 4: note = MISC_FEATURE - Xaa is de
GXXXSSC

SEQ ID NO: 247-253 - skipped (7 entries)